European Patent Application EP 4 116 328 A1, published January 11, 2023. Title: COMBINATION THERAPIES TARGETING PD-1, TIM-3, AND LAG-3. Applicant: SYMPHOGEN A/S. Application Not yet assigned. The sequence listing filed with the application follows.

SEQUENCE LISTING (397 sequences)

SEQ ID NO: 1 - DNA, 360 bp, Artificial Sequence
  source: /note="Description of Artificial Sequence: Synthetic polynucleotide"
caggtgcagctacagcagtcgggcccaggactggtgaagccttcacagaccctgtccctcacctgcactgtctctggtggctccatcagcagtggtggttactactggagttggacccgtcagcacccagggatgggcctggagtggattggatacatctcttacagtgggagtatctattacactccgtccctcaagagtcgacttaccatatcagtggacacgtctaagaaccagttctccctgaagctgagctctgtgactgccgcggacacggccgtatattactgtgcgagtttggattcctggggatctaaccgtgactactggggccagggaaccctggtcaccgtctcgagt

SEQ ID NO: 2 - DNA, 321 bp, Artificial Sequence
  source: /note="Description of Artificial Sequence: Synthetic polynucleotide"
gaaattgtgttgacgcagtctccagccaccctgtctttgtctccaggggaaagagccaccctctcctgcagggccagtcagagtgttagcagctacttagcctggtaccaacagaaacctggccaggctcccaggctcctcatctatgatgcatccaacagggccactggcatcccagccaggttcagtggcagtgggtctgggacagacttcactctcaccatcagcagcctagagcctgaagattttgcagtttattactgtcagcagcgtagcaactggccgctcactttcggcggagggaccaaggtggagattaag

SEQ ID NO: 3 - protein, 120 aa, Artificial Sequence
  source: /note="Description of Artificial Sequence: Synthetic polypeptide"
QVQLQQSGPGLVKPSQTLSLTCTVSGGSISSGGYYWSWTRQHPGMGLEWIGYISYSGSIYYTPSLKSRLTISVDTSKNQFSLKLSSVTAADTAVYYCASLDSWGSNRDYWGQGTLVTVSS

SEQ ID NO: 4 - protein, 107 aa, Artificial Sequence
  source: /note="Description of Artificial Sequence: Synthetic polypeptide"
EIVLTQSPATLSLSPGERATLSCRASQSVSSYLAWYQQKPGQAPRLLIYDASNRATGIPARFSGSGSGTDFTLTISSLEPEDFAVYYCQQRSNWPLTFGGGTKVEIK

SEQ ID NO: 5 - DNA, 360 bp, Artificial Sequence
  source: /note="Description of Artificial Sequence: Synthetic polynucleotide"
caggtgcagctgcaggagagtggccccggactggtcaagccttcacagactctgagcctgacctgcacagtgtctggcggaagtatcagctccgggggttactattggagctggacccgacagcacccaggaatgggtctggaatggatcgggtacatttcatatagcggctccatctactatacaccctcactgaaaagcaggctgaccatttccgtggacacatctaagaaccagttcagcctgaaactgtctagtgtgacagccgctgatactgcagtctactattgtgcctccctggactcttggggcagtaatagagattactggggccagggaactctggtcaccgtctcgagt

SEQ ID NO: 6 - DNA, 321 bp, Artificial Sequence
  source: /note="Description of Artificial Sequence: Synthetic polynucleotide"
gagatcgtgctgactcagtccccagccaccctgtcactgagcccaggagaacgagcaaccctgtcttgcagggcctcccagtctgtcagctcctacctggcttggtatcagcagaagcccgggcaggcacctcgactgctgatctacgacgccagtaacagagctaccggtattcccgcccgcttcagtggttcaggcagcggaacagactttaccctgacaatctctagtctggagcctgaagatttcgccgtgtactattgtcagcagaggtctaattggccactgacatttggcggagggactaaggtcgagatcaag

SEQ ID NO: 7 - protein, 120 aa, Artificial Sequence
  source: /note="Description of Artificial Sequence: Synthetic polypeptide"
QVQLQESGPGLVKPSQTLSLTCTVSGGSISSGGYYWSWTRQHPGMGLEWIGYISYSGSIYYTPSLKSRLTISVDTSKNQFSLKLSSVTAADTAVYYCASLDSWGSNRDYWGQGTLVTVSS

SEQ ID NO: 8 - protein, 10 aa, Artificial Sequence
  source: /note="Description of Artificial Sequence: Synthetic peptide"
GGSISSGGYY

SEQ ID NO: 9 - protein, 7 aa, Artificial Sequence
  source: /note="Description of Artificial Sequence: Synthetic peptide"
ISYSGSI

SEQ ID NO: 10 - protein, 14 aa, Artificial Sequence
  source: /note="Description of Artificial Sequence: Synthetic peptide"
CASLDSWGSNRDYW

SEQ ID NO: 11 - protein, 6 aa, Artificial Sequence
  source: /note="Description of Artificial Sequence: Synthetic peptide"
QSVSSY

SEQ ID NO: 12 - protein, 3 aa, Artificial Sequence
  source: /note="Description of Artificial Sequence: Synthetic peptide"
DAS

SEQ ID NO: 13 - protein, 11 aa, Artificial Sequence [sequence omitted]

SEQ ID NO: 14 - DNA, 345 bp, Artificial Sequence
  source: /note="Description of Artificial Sequence: Synthetic polynucleotide"
caggtcaccttgaaggagtggggcgcaggactgttgaggccctcggagaccctgtccctcacctgcgctgtctatggtgggtccttcagtggttactactggagctggatccgccagcccccagggaaggggctggagtggataggggaaatcaatcatagtggaagcaccaactacaacccgtccctcaagagtcgagtcaccatatcagtagacgcgaccaagaaacaattctccctgaagctgacctctgtgaccgccgcggacacggctgtgtattactgtgcgagatattgggagctccctgactactggggccagggcaccctggtcaccgtctcgagt

SEQ ID NO: 15 - DNA, 321 bp, Artificial Sequence
  source: /note="Description of Artificial Sequence: Synthetic polynucleotide"
gacatccagttgacccagtctccatcctccctgtctgcatctgtaggagacagagtcaccatcacttgccgggcaagtcagggcattagaaatgatttaggctggtatcagcagaaaccagggaaagcccctaagcgcctgatctatgctgcatccagtttgcaaagtggggtcccatcaaggttcagcggcagtggatctgggacagaattcactctcacaatcagcagcctgcagcctgaagattttgcaacttattactgtctacagcataatagttaccctccgacgttcggccaagggaccaaggtggaaatcaag

SEQ ID NO: 16 - protein, 115 aa, Artificial Sequence
  source: /note="Description of Artificial Sequence: Synthetic polypeptide"
QVTLKEWGAGLLRPSETLSLTCAVYGGSFSGYYWSWIRQPPGKGLEWIGEINHSGSTNYNPSLKSRVTISVDATKKQFSLKLTSVTAADTAVYYCARYWELPDYWGQGTLVTVSS

SEQ ID NO: 17 - protein, 107 aa, Artificial Sequence
  source: /note="Description of Artificial Sequence: Synthetic polypeptide"
DIQLTQSPSSLSASVGDRVTITCRASQGIRNDLGWYQQKPGKAPKRLIYAASSLQSGVPSRFSGSGSGTEFTLTISSLQPEDFATYYCLQHNSYPPTFGQGTKVEIK

SEQ ID NO: 18 - protein, 8 aa, Artificial Sequence
  source: /note="Description of Artificial Sequence: Synthetic peptide"
GGSFSGYY

SEQ ID NO: 19 - protein, 7 aa, Artificial Sequence
  source: /note="Description of Artificial Sequence: Synthetic peptide"
INHSGST

SEQ ID NO: 20 - protein, 11 aa, Artificial Sequence
  source: /note="Description of Artificial Sequence: Synthetic peptide"
CARYWELPDYW

SEQ ID NO: 21 - protein, 6 aa, Artificial Sequence
  source: /note="Description of Artificial Sequence: Synthetic peptide"
QGIRND

SEQ ID NO: 22 - protein, 3 aa, Artificial Sequence
  source: /note="Description of Artificial Sequence: Synthetic peptide"
AAS

SEQ ID NO: 23 - protein, 11 aa, Artificial Sequence [sequence omitted]

SEQ ID NO: 24 - DNA, 345 bp, Artificial Sequence
  source: /note="Description of Artificial Sequence: Synthetic polynucleotide"
cagatgcagctggtgcagtggggcgcaggactgttgaagccttcggagaccctgtccctcacctgcgctgtctatggtgggtccttcagtggttactactggagctggatccgccagcccccagggaaggggctggagtggattggggaaatcaatcatagtggaagcaccaactacaacccgtccctcaagagtcgagtcaccatgtcagttgacacgtccaagcaccagttctccctgaagctgagctctgtgaccgccgcggacacggctgtgtattactgtgcgagatggtgggagcttcctgactactggggccagggaaccctggtcaccgtctcgagt

SEQ ID NO: 25 - DNA, 321 bp, Artificial Sequence
  source: /note="Description of Artificial Sequence: Synthetic polynucleotide"
gaaattgtgttgacgcagtctccatcctccctgtctgcatctgtaggagacagagtcaccatcacttgccgggcaagtcagggcattagaaatgatttaggctggtatcagcagaaaccagggaaagcccctaagcgcctgatctatgctgcatccagtttgcaaagtggggtcccatcaaggttcagcggcagtggatctgggacagaattcactctcacaatcagcagcctgcagcctgaagattttgcaacttattactgtctacagcataatagttacccgtggacgttcggccaagggaccaaggtggaaatcaag

SEQ ID NO: 26 - protein, 115 aa, Artificial Sequence
  source: /note="Description of Artificial Sequence: Synthetic polypeptide"
QMQLVQWGAGLLKPSETLSLTCAVYGGSFSGYYWSWIRQPPGKGLEWIGEINHSGSTNYNPSLKSRVTMSVDTSKHQFSLKLSSVTAADTAVYYCARWWELPDYWGQGTLVTVSS

SEQ ID NO: 27 - protein, 107 aa, Artificial Sequence
  source: /note="Description of Artificial Sequence: Synthetic polypeptide"
EIVLTQSPSSLSASVGDRVTITCRASQGIRNDLGWYQQKPGKAPKRLIYAASSLQSGVPSRFSGSGSGTEFTLTISSLQPEDFATYYCLQHNSYPWTFGQGTKVEIK

SEQ ID NO: 28 - protein, 8 aa, Artificial Sequence
  source: /note="Description of Artificial Sequence: Synthetic peptide"
GGSFSGYY

SEQ ID NO: 29 - protein, 7 aa, Artificial Sequence
  source: /note="Description of Artificial Sequence: Synthetic peptide"
INHSGST

SEQ ID NO: 30 - protein, 11 aa, Artificial Sequence
  source: /note="Description of Artificial Sequence: Synthetic peptide"
CARWWELPDYW

SEQ ID NO: 31 - protein, 6 aa, Artificial Sequence
  source: /note="Description of Artificial Sequence: Synthetic peptide"
QGIRND

SEQ ID NO: 32 - protein, 3 aa, Artificial Sequence
  source: /note="Description of Artificial Sequence: Synthetic peptide"
AAS

SEQ ID NO: 33 - protein, 11 aa, Artificial Sequence [sequence omitted]

SEQ ID NO: 34 - DNA, 351 bp, Artificial Sequence
  source: /note="Description of Artificial Sequence: Synthetic polynucleotide"
cagatgcagctggtgcaatggggcgcaggactgttgaagccttcggagaccctgtccctcacctgcgctgtctatggtgggtccttcagtggttactactggagctggatccgccagcccccagggaaggggctggagtggattggggaaatcaatcatagtggaagcaccaactacaacccgtccctcaagagtcgagtcaccatatcagtagacacgtccaagaaccagttctccctgaagctgagctctgtgaccgccgcggacacggctgtgtattactgtgcgaggttttactatgctccgaactttgactactggggccagggcaccctggtcaccgtctcgagt

SEQ ID NO: 35 - DNA, 318 bp, Artificial Sequence
  source: /note="Description of Artificial Sequence: Synthetic polynucleotide"
gaaattgtgttgacgcagtctccttccaccctgtctgcatctgtaggagacagagtcaccatcacttgccgggccagtcagagtattagtagctggttggcctggtatcagcagaaaccagggacagcccctaagctcctgatctataaggcgtctagtttagaaagtggggtcccatcaaggttcagcggcagtggatctgggacagaattcactctcaccatcagcagcctgcagcctgatgattttgcaacttattactgccaacagtataatagttattccactttcggcggagggaccaaggtggagatcaaa

SEQ ID NO: 36 - protein, 117 aa, Artificial Sequence
  source: /note="Description of Artificial Sequence: Synthetic polypeptide"
QMQLVQWGAGLLKPSETLSLTCAVYGGSFSGYYWSWIRQPPGKGLEWIGEINHSGSTNYNPSLKSRVTISVDTSKNQFSLKLSSVTAADTAVYYCARFYYAPNFDYWGQGTLVTVSS

SEQ ID NO: 37 - protein, 106 aa, Artificial Sequence
  source: /note="Description of Artificial Sequence: Synthetic polypeptide"
EIVLTQSPSTLSASVGDRVTITCRASQSISSWLAWYQQKPGTAPKLLIYKASSLESGVPSRFSGSGSGTEFTLTISSLQPDDFATYYCQQYNSYSTFGGGTKVEIK

SEQ ID NO: 38 - protein, 8 aa, Artificial Sequence
  source: /note="Description of Artificial Sequence: Synthetic peptide"
GGSFSGYY

SEQ ID NO: 39 - protein, 7 aa, Artificial Sequence
  source: /note="Description of Artificial Sequence: Synthetic peptide"
INHSGST

SEQ ID NO: 40 - protein, 13 aa, Artificial Sequence
  source: /note="Description of Artificial Sequence: Synthetic peptide"
CARFYYAPNFDYW

SEQ ID NO: 41 - protein, 6 aa, Artificial Sequence
  source: /note="Description of Artificial Sequence: Synthetic peptide"
QSISSW

SEQ ID NO: 42 - protein, 3 aa, Artificial Sequence
  source: /note="Description of Artificial Sequence: Synthetic peptide"
KAS

SEQ ID NO: 43 - protein, 10 aa, Artificial Sequence [sequence omitted]

SEQ ID NO: 44 - DNA, 360 bp, Artificial Sequence
  source: /note="Description of Artificial Sequence: Synthetic polynucleotide"
caggtgcagctgcagcagtcgggcccaggactggtgaagccttcggagaccctgtccctcacctgcactgtctctggtggctccatcagcagtagtaattactactggggctggatccgccagcccccagggaaggggctggagtggattgggagtatctattatagtgggaacacctactacaacccgtccctcaagagtcgagtcaccatatccgtagacacgtccaagaaccagttctccctgaagctgagttctgtgaccgccgcagacacggctgtgtattactgtgcgagacagacagtggctggccccctctttgactactggggccagggaaccctggtcaccgtctcgagt

SEQ ID NO: 45 - DNA, 321 bp, Artificial Sequence
  source: /note="Description of Artificial Sequence: Synthetic polynucleotide"
gaaattgtgatgacgcagtctccttccaccctgtctgcatctgtaggagacagagtcaccatcacttgccgggccagtcagagtattagtagctggttggcctggtatcagcagaaaccagggaaagcccctaaggtcctgatctataaggcgtctagtttagaaagtggggtcccatcaaggttcagcggcagtggatctgggacagaactcactctcaccatcagcagcctgcagcctgatgattttgcaacttattactgccaacagtataatagttattcattcactttcggccctgggaccaaagtggatatcaag

SEQ ID NO: 46 - protein, 120 aa, Artificial Sequence
  source: /note="Description of Artificial Sequence: Synthetic polypeptide"
QVQLQQSGPGLVKPSETLSLTCTVSGGSISSSNYYWGWIRQPPGKGLEWIGSIYYSGNTYYNPSLKSRVTISVDTSKNQFSLKLSSVTAADTAVYYCARQTVAGPLFDYWGQGTLVTVSS

SEQ ID NO: 47 - protein, 107 aa, Artificial Sequence
  source: /note="Description of Artificial Sequence: Synthetic polypeptide"
EIVMTQSPSTLSASVGDRVTITCRASQSISSWLAWYQQKPGKAPKVLIYKASSLESGVPSRFSGSGSGTELTLTISSLQPDDFATYYCQQYNSYSFTFGPGTKVDIK

SEQ ID NO: 48 - protein, 10 aa, Artificial Sequence
  source: /note="Description of Artificial Sequence: Synthetic peptide"
GGSISSSNYY

SEQ ID NO: 49 - protein, 7 aa, Artificial Sequence
  source: /note="Description of Artificial Sequence: Synthetic peptide"
IYYSGNT

SEQ ID NO: 50 - protein, 14 aa, Artificial Sequence
  source: /note="Description of Artificial Sequence: Synthetic peptide"
CARQTVAGPLFDYW

SEQ ID NO: 51 - protein, 6 aa, Artificial Sequence
  source: /note="Description of Artificial Sequence: Synthetic peptide"
QSISSW

SEQ ID NO: 52 - protein, 3 aa, Artificial Sequence
  source: /note="Description of Artificial Sequence: Synthetic peptide"
KAS

SEQ ID NO: 53 - protein, 11 aa, Artificial Sequence [sequence omitted]

SEQ ID NO: 54 - DNA, 375 bp, Artificial Sequence
  source: /note="Description of Artificial Sequence: Synthetic polynucleotide"
caggtccagctggtgcaatctggggctgaggtgaagaagcctggggcctcagtgaaggtctcctgcaaggctgctggatacaccttaaccggctactatatgcactgggtgcgacaggcccctggacaaggccttgagtggatgggacggatcaaccctaacagtggtggctcaaacaatgcacagaagtttcagggcagggtcaccatgaccagggacacgtccatcagcacagcctacatggagctgagcaggctgagatctgacgacacggccgtgtattactgtgcgagagagggtcccctgtatagcagtggctggtacgagggtgcttttgatatctggggccaagggacaatggtcaccgtctcgagt

SEQ ID NO: 55 - DNA, 327 bp, Artificial Sequence
  source: /note="Description of Artificial Sequence: Synthetic polynucleotide"
gaaattgtgatgacgcagtctccttccaccctgtctgcatctgtaggagacagagtcaccatcacttgccgggccagtcagagtattagtagttggttggcctggtatcagcagaaaccagggaaagcccctaagctcctgatctataaggcgtctagtttagaaagtggggtcccatcaaggttcagcggcagtggatctgggacagaattcactctcaccatcagcagcctgcagcctgatgattttgcaacttattactgccaacagtataatagttattctccggggctcactttcggcggagggaccaaggtggagatcaag

SEQ ID NO: 56 - protein, 125 aa, Artificial Sequence
  source: /note="Description of Artificial Sequence: Synthetic polypeptide"
QVQLVQSGAEVKKPGASVKVSCKAAGYTLTGYYMHWVRQAPGQGLEWMGRINPNSGGSNNAQKFQGRVTMTRDTSISTAYMELSRLRSDDTAVYYCAREGPLYSSGWYEGAFDIWGQGTMVTVSS

SEQ ID NO: 57 - protein, 109 aa, Artificial Sequence
  source: /note="Description of Artificial Sequence: Synthetic polypeptide"
EIVMTQSPSTLSASVGDRVTITCRASQSISSWLAWYQQKPGKAPKLLIYKASSLESGVPSRFSGSGSGTEFTLTISSLQPDDFATYYCQQYNSYSPGLTFGGGTKVEIK

SEQ ID NO: 58 - protein, 8 aa, Artificial Sequence
  source: /note="Description of Artificial Sequence: Synthetic peptide"
GYTLTGYY

SEQ ID NO: 59 - protein, 8 aa, Artificial Sequence
  source: /note="Description of Artificial Sequence: Synthetic peptide"
INPNSGGS

SEQ ID NO: 60 - protein, 20 aa, Artificial Sequence
  source: /note="Description of Artificial Sequence: Synthetic peptide"
CAREGPLYSSGWYEGAFDIW

SEQ ID NO: 61 - protein, 6 aa, Artificial Sequence
  source: /note="Description of Artificial Sequence: Synthetic peptide"
QSISSW

SEQ ID NO: 62 - protein, 3 aa, Artificial Sequence
  source: /note="Description of Artificial Sequence: Synthetic peptide"
KAS

SEQ ID NO: 63 - protein, 13 aa, Artificial Sequence [sequence omitted]

SEQ ID NO: 64 - DNA, 372 bp, Artificial Sequence
  source: /note="Description of Artificial Sequence: Synthetic polynucleotide"
cagatgcagctacagcagtcaggtccaggactggtgaagccctcgcagaccctctcactcacctgtgccatctccggggacagtgtctctagcaacagtgctgcttggaactggatcaggcagtccccatcgagaggccttgagtggctgggaaggacatactacaggtccaagtggtattctgcttttgcagtatctgtgaaaagtcgaataaccatcaacccagacacatccaagaaccagttctccctgcagctgaactctgtgactcccgaggacacggctgtgtattactgtgcaagagagggtagcagtggctggtacggatacgtccaccactggggccagggcaccctggtcaccgtctcgagt

SEQ ID NO: 65 - DNA, 321 bp, Artificial Sequence
  source: /note="Description of Artificial Sequence: Synthetic polynucleotide"
gaaattgtgttgacgcagtctccagcttccctgtctgtatctctgggagaaactgtcaccatcgaatgtcgagcaagtgaggacatttacaatggtttagcatggtatcagcagaagccagggaaatctcctcagctcctgatctataatgcaaatagcttgcatactggggtcccatcacggttcagtggcagtggatctggtacacagtattctctcaagataaacagcctgcaatctgaagatgtcgcaagttatttctgtcaacagtattacgattatcctccgacgttcggccaagggaccaaggtggaaatcaaa

SEQ ID NO: 66 - protein, 124 aa, Artificial Sequence
  source: /note="Description of Artificial Sequence: Synthetic polypeptide"
QMQLQQSGPGLVKPSQTLSLTCAISGDSVSSNSAAWNWIRQSPSRGLEWLGRTYYRSKWYSAFAVSVKSRITINPDTSKNQFSLQLNSVTPEDTAVYYCAREGSSGWYGYVHHWGQGTLVTVSS

SEQ ID NO: 67 - protein, 107 aa, Artificial Sequence
  source: /note="Description of Artificial Sequence: Synthetic polypeptide"
EIVLTQSPASLSVSLGETVTIECRASEDIYNGLAWYQQKPGKSPQLLIYNANSLHTGVPSRFSGSGSGTQYSLKINSLQSEDVASYFCQQYYDYPPTFGQGTKVEIK

SEQ ID NO: 68 - protein, 10 aa, Artificial Sequence
  source: /note="Description of Artificial Sequence: Synthetic peptide"
GDSVSSNSAA

SEQ ID NO: 69 - protein, 9 aa, Artificial Sequence
  source: /note="Description of Artificial Sequence: Synthetic peptide"
TYYRSKWYS

SEQ ID NO: 70 - protein, 16 aa, Artificial Sequence
  source: /note="Description of Artificial Sequence: Synthetic peptide"
CAREGSSGWYGYVHHW

SEQ ID NO: 71 - protein, 6 aa, Artificial Sequence
  source: /note="Description of Artificial Sequence: Synthetic peptide"
EDIYNG

SEQ ID NO: 72 - protein, 3 aa, Artificial Sequence
  source: /note="Description of Artificial Sequence: Synthetic peptide"
NAN

SEQ ID NO: 73 - protein, 11 aa, Artificial Sequence
  source: /note="Description of Artificial Sequence: Synthetic peptide"
CQQYYDYPPTF

SEQ ID NO: 74 - DNA, 369 bp, Artificial Sequence
  source: /note="Description of Artificial Sequence: Synthetic polynucleotide"
caggtgcagctgcaggagtcgggcccaggactggtgaagccttcggagaccctgtccctcacctgcactgtctctggtggctccttcagcagtagtagttactactggggctggatccgccagccccctgggaaggggctggagtggattgggatcttctattatagtgggaccacctactacaacccgtccctcaagagtcgagtcaccatatccgcacacacgtccaagagccagttctccctgaagctgagctctgtgaccgccgcagacacggctgtgtattactgtgcgagagggggagaatattttgaccggttactcccctttgactactggggccagggaaccctggtcaccgtctcgagt

SEQ ID NO: 75 - DNA, 321 bp, Artificial Sequence
  source: /note="Description of Artificial Sequence: Synthetic polynucleotide"
gaaattgtgatgacgcagtctccatccttcctgtctgcatctgtaggagacagagtcaccatcacttgccgggccagtcagggcattagcagttatttagcctggtatcagcaaaaaccagggaaagcccctaagctcctgatctatgctgcatccactttggaaagtggggtcccatcaaggttcagcggcagtggatctgggacagaattcactctcacaatcagcagcctgcagcctgaagattttgcaacttattactgtcaacagcttaatagttacccattcactttcggccctgggaccaaagtggatatcaaa

SEQ ID NO: 76 - protein, 123 aa, Artificial Sequence
  source: /note="Description of Artificial Sequence: Synthetic polypeptide"
QVQLQESGPGLVKPSETLSLTCTVSGGSFSSSSYYWGWIRQPPGKGLEWIGIFYYSGTTYYNPSLKSRVTISAHTSKSQFSLKLSSVTAADTAVYYCARGGEYFDRLLPFDYWGQGTLVTVSS

SEQ ID NO: 77 - protein, 107 aa, Artificial Sequence
  source: /note="Description of Artificial Sequence: Synthetic polypeptide"
EIVMTQSPSFLSASVGDRVTITCRASQGISSYLAWYQQKPGKAPKLLIYAASTLESGVPSRFSGSGSGTEFTLTISSLQPEDFATYYCQQLNSYPFTFGPGTKVDIK

SEQ ID NO: 78 - protein, 10 aa, Artificial Sequence
  source: /note="Description of Artificial Sequence: Synthetic peptide"
GGSFSSSSYY

SEQ ID NO: 79 - protein, 7 aa, Artificial Sequence
  source: /note="Description of Artificial Sequence: Synthetic peptide"
FYYSGTT

SEQ ID NO: 80 - protein, 17 aa, Artificial Sequence
  source: /note="Description of Artificial Sequence: Synthetic peptide"
CARGGEYFDRLLPFDYW

SEQ ID NO: 81 - protein, 6 aa, Artificial Sequence
  source: /note="Description of Artificial Sequence: Synthetic peptide"
QGISSY

SEQ ID NO: 82 - protein, 3 aa, Artificial Sequence
  source: /note="Description of Artificial Sequence: Synthetic peptide"
AAS

SEQ ID NO: 83 - protein, 11 aa, Artificial Sequence [sequence omitted]

SEQ ID NO: 84 - DNA, 351 bp, Artificial Sequence
  source: /note="Description of Artificial Sequence: Synthetic polynucleotide"
caggtgcagctggtggagtctgggggaggcttggtacagccgggggggtccctgagactctcctgtacagcctctggattcacctttagcagctatgccatgagctgggtccgccaggctccagggaaggggctggagtgggtctcagctattggtggtagtggtggtagcacatactacgcagactccgtgaagggccggttcaccatctccagagacaattccaagaacacgctgtatctgcaaatgaacagcctgagagccgaggacacggccgtatattactgtgtgaaagatggggcaggaggctttgactactggggccagggaaccctggtcaccgtctcgagt

SEQ ID NO: 85 - DNA, 321 bp, Artificial Sequence
  source: /note="Description of Artificial Sequence: Synthetic polynucleotide"
gatattgtgatgacgcagtcttcatcctccctgtctgcatctgtaggagacagagtcaccatcacttgccgggcaagtcagggcattataaatcatttaggctggtatcagcataaaccagggaaagcccctaatcgcctaatctatgctgcatccagtttgcaaagtggggtcccatcaaggttcagcggcagtggatctgggacagaattcactctcacaatcagcagcctgcagcctgaagattttgcaacttattactgtctacggcataatagttaccctccgacgttcggccaagggaccaaggtggaaatcaag

SEQ ID NO: 86 - protein, 117 aa, Artificial Sequence
  source: /note="Description of Artificial Sequence: Synthetic polypeptide"
QVQLVESGGGLVQPGGSLRLSCTASGFTFSSYAMSWVRQAPGKGLEWVSAIGGSGGSTYYADSVKGRFTISRDNSKNTLYLQMNSLRAEDTAVYYCVKDGAGGFDYWGQGTLVTVSS

SEQ ID NO: 87 - protein, 107 aa, Artificial Sequence
  source: /note="Description of Artificial Sequence: Synthetic polypeptide"
DIVMTQSSSSLSASVGDRVTITCRASQGIINHLGWYQHKPGKAPNRLIYAASSLQSGVPSRFSGSGSGTEFTLTISSLQPEDFATYYCLRHNSYPPTFGQGTKVEIK

SEQ ID NO: 88 - protein, 8 aa, Artificial Sequence
  source: /note="Description of Artificial Sequence: Synthetic peptide"
GFTFSSYA

SEQ ID NO: 89 - protein, 8 aa, Artificial Sequence
  source: /note="Description of Artificial Sequence: Synthetic peptide"
IGGSGGST

SEQ ID NO: 90 - protein, 12 aa, Artificial Sequence
  source: /note="Description of Artificial Sequence: Synthetic peptide"
CVKDGAGGFDYW

SEQ ID NO: 91 - protein, 6 aa, Artificial Sequence
  source: /note="Description of Artificial Sequence: Synthetic peptide"
QGIINH

SEQ ID NO: 92 - protein, 3 aa, Artificial Sequence
  source: /note="Description of Artificial Sequence: Synthetic peptide"
AAS

SEQ ID NO: 93 - protein, 5 aa, Artificial Sequence
  source: /note="Description of Artificial Sequence: Synthetic peptide"
YPPTF

SEQ ID NO: 94 - DNA, 366 bp, Artificial Sequence
  source: /note="Description of Artificial Sequence: Synthetic polynucleotide"
caggtgcagctacagcagtcgggcccaggactggtgaagccttcacagaccctgtccctcacctgcactgtctctggtggctccatcaacagtggtggtcactactggagctggatccgccagcacccagggaggggcctggagtggattgggtacatctattacagtgggagcatctactacaacccgtccctcaagagtcgacttaccatatcagtagacacgtctaagaaccagttctccctgaagctgagctctgtgactgccgcggacacggccgtgtattactgtgcgagttattactatgccagtagtggtgatgcttttgatatctggggccaagggacaatggtcaccgtctcgagt

SEQ ID NO: 95 - DNA, 321 bp, Artificial Sequence
  source: /note="Description of Artificial Sequence: Synthetic polynucleotide"
gaaacgacactcacgcagtctccagccaccctgtctttgtctccaggggaaagagccaccctctcctgcagggccagtcagagtgttagcagctacttagcctggtaccaacagaaacctggccaggctcccaggctcctcatctatgatgcatccaacagggccactggcatcccagccaggttcagtggcagtgggtctgggacagacttcactctcaccatcagcagcctagagcctgaagattttgcagtttattactgtcagcagcgtagcaactggcctccgacgttcggccaagggaccaaggtggaaatcaaa

SEQ ID NO: 96 - protein, 122 aa, Artificial Sequence
  source: /note="Description of Artificial Sequence: Synthetic polypeptide"
QVQLQQSGPGLVKPSQTLSLTCTVSGGSINSGGHYWSWIRQHPGRGLEWIGYIYYSGSIYYNPSLKSRLTISVDTSKNQFSLKLSSVTAADTAVYYCASYYYASSGDAFDIWGQGTMVTVSS

SEQ ID NO: 97 - protein, 107 aa, Artificial Sequence
  source: /note="Description of Artificial Sequence: Synthetic polypeptide"
ETTLTQSPATLSLSPGERATLSCRASQSVSSYLAWYQQKPGQAPRLLIYDASNRATGIPARFSGSGSGTDFTLTISSLEPEDFAVYYCQQRSNWPPTFGQGTKVEIK

SEQ ID NO: 98 - protein, 10 aa, Artificial Sequence
  source: /note="Description of Artificial Sequence: Synthetic peptide"
GGSINSGGHY

SEQ ID NO: 99 - protein, 7 aa, Artificial Sequence
  source: /note="Description of Artificial Sequence: Synthetic peptide"
IYYSGSI

SEQ ID NO: 100 - protein, 16 aa, Artificial Sequence
  source: /note="Description of Artificial Sequence: Synthetic peptide"
CASYYYASSGDAFDIW

SEQ ID NO: 101 - protein, 6 aa, Artificial Sequence
  source: /note="Description of Artificial Sequence: Synthetic peptide"
QSVSSY

SEQ ID NO: 102 - protein, 3 aa, Artificial Sequence
  source: /note="Description of Artificial Sequence: Synthetic peptide"
DAS

SEQ ID NO: 103 - protein, 11 aa, Artificial Sequence [sequence omitted]

SEQ ID NO: 104 - DNA, 372 bp, Artificial Sequence
  source: /note="Description of Artificial Sequence: Synthetic polynucleotide"
caggtgcagctgcaggagtctgggggaggcttggtacagccgggggggtccctgagactctcctgtacagcctctggattcacctttagtaattatgccatgagctgggtccgccaggctccagggaaggggctggagtgggtctcagctattagtggtcgtggtggtagcacattcttcgcagactccgtgaagggccggttcaccatctccagagacaattccaagagcacgctgtatctgcaaacgaacagcctgagagccgaggacacggccgtatattactgtgcgaaagggggcccgttgtataactggaacgacggtgatggttttgatatctggggccaagggaccacggtcacagtctcgagt

SEQ ID NO: 105 - DNA, 324 bp, Artificial Sequence
  source: /note="Description of Artificial Sequence: Synthetic polynucleotide"
gaaattgtgttgacgcagtctccagccaccctgtctgtgtctccaggggaaagagccaccctctcctgcagggccagtcagagtgttagcagcaacttagcctggtaccagcagaaacctggccaggctcccaggctcctcatctatggtgcatccaccagggccactggtatcccagccaggttcagtggcactgggtctgggacagagttcactctcaccatcagcagcctgcagtctgaagattttgcactttattactgtcagcagtatgataactggcctccgtggacgttcggccaagggaccaaggtggaaatcaaa

SEQ ID NO: 106 - protein, 124 aa, Artificial Sequence
  source: /note="Description of Artificial Sequence: Synthetic polypeptide"
QVQLQESGGGLVQPGGSLRLSCTASGFTFSNYAMSWVRQAPGKGLEWVSAISGRGGSTFFADSVKGRFTISRDNSKSTLYLQTNSLRAEDTAVYYCAKGGPLYNWNDGDGFDIWGQGTTVTVSS

SEQ ID NO: 107 - protein, 108 aa, Artificial Sequence
  source: /note="Description of Artificial Sequence: Synthetic polypeptide"
EIVLTQSPATLSVSPGERATLSCRASQSVSSNLAWYQQKPGQAPRLLIYGASTRATGIPARFSGTGSGTEFTLTISSLQSEDFALYYCQQYDNWPPWTFGQGTKVEIK

SEQ ID NO: 108 - protein, 8 aa, Artificial Sequence
  source: /note="Description of Artificial Sequence: Synthetic peptide"
GFTFSNYA

SEQ ID NO: 109 - protein, 8 aa, Artificial Sequence
  source: /note="Description of Artificial Sequence: Synthetic peptide"
ISGRGGST

SEQ ID NO: 110 - protein, 19 aa, Artificial Sequence
  source: /note="Description of Artificial Sequence: Synthetic peptide"
CAKGGPLYNWNDGDGFDIW

SEQ ID NO: 111 - protein, 6 aa, Artificial Sequence
  source: /note="Description of Artificial Sequence: Synthetic peptide"
QSVSSN

SEQ ID NO: 112 - protein, 3 aa, Artificial Sequence
  source: /note="Description of Artificial Sequence: Synthetic peptide"
GAS

SEQ ID NO: 113 - protein, 12 aa, Artificial Sequence [sequence omitted]

SEQ ID NO: 114 - DNA, 357 bp, Artificial Sequence
  source: /note="Description of Artificial Sequence: Synthetic polynucleotide"
caggtgcagctgcaggagtctgggggaggcttggtcaagcctggagggtccctgagactctcctgtgcagcctctggattcaccttcagtgactactacatgacctggatccgccaggctccagggaaggggctggagtggatttcatacattagtggtggtggtggttccatatactacgcagactctgtgaagggccgattcaccatctccagggacaacgccaagaactcactgtatctgcaaatgaacagcctgagagccgaggacacggccgtttatttctgtgcgagagggaactggggatcggcggctcttgatatctggggccaagggacaatggtcacggtctcgagt

SEQ ID NO: 115 - DNA, 321 bp, Artificial Sequence
  source: /note="Description of Artificial Sequence: Synthetic polynucleotide"
gaaattgtgttgacgcagtctccatcctcactgtctgcatctgtaggagacagagtcaccatcacttgtcgggcgagtcagggcattaacaattatttagcctggtttcagcagaaaccagggagagcccctaagtccctgatctatgctgcatccagtttgcaaagtggggtcccatcgaagttcagcggcagtggatctgggacagatttcactctcaccatcagcagcctgcagcctgaagattttgcaacttattactgccaacagtataatagttaccctccaactctcggccctgggaccaacgtggatatcaaa

SEQ ID NO: 116 - protein, 119 aa, Artificial Sequence
  source: /note="Description of Artificial Sequence: Synthetic polypeptide"
QVQLQESGGGLVKPGGSLRLSCAASGFTFSDYYMTWIRQAPGKGLEWISYISGGGGSIYYADSVKGRFTISRDNAKNSLYLQMNSLRAEDTAVYFCARGNWGSAALDIWGQGTMVTVSS

SEQ ID NO: 117 - protein, 107 aa, Artificial Sequence
  source: /note="Description of Artificial Sequence: Synthetic polypeptide"
EIVLTQSPSSLSASVGDRVTITCRASQGINNYLAWFQQKPGRAPKSLIYAASSLQSGVPSKFSGSGSGTDFTLTISSLQPEDFATYYCQQYNSYPPTLGPGTNVDIK

SEQ ID NO: 118 - protein, 8 aa, Artificial Sequence
  source: /note="Description of Artificial Sequence: Synthetic peptide"
GFTFSDYY

SEQ ID NO: 119 - protein, 11 aa, Artificial Sequence
  source: /note="Description of Artificial Sequence: Synthetic peptide"
ISYISGGGGSI

SEQ ID NO: 120 - protein, 14 aa, Artificial Sequence
  source: /note="Description of Artificial Sequence: Synthetic peptide"
CARGNWGSAALDIW

SEQ ID NO: 121 - protein, 6 aa, Artificial Sequence
  source: /note="Description of Artificial Sequence: Synthetic peptide"
QGINNY

SEQ ID NO: 122 - protein, 3 aa, Artificial Sequence
  source: /note="Description of Artificial Sequence: Synthetic peptide"
AAS

SEQ ID NO: 123 - protein, 11 aa, Artificial Sequence
  source: /note="Description of Artificial Sequence: Synthetic peptide"
CQQYNSYPPTL

SEQ ID NO: 124 - DNA, 351 bp, Artificial Sequence
  source: /note="Description of Artificial Sequence: Synthetic polynucleotide"
caggtgcagctggtggagtctgggggaggcttggtacagccgggggggtccctgagactctcctgtacagcctctggattcacctttagcagctatgccatgagctgggtccgccaggctccagggaaggggctggagtgggtctcagctattggtggtagtggtggtagcgcatactacgcagactccgtgaagggccggttcaccatctccagagacaattccaagaacacgctgtatctgcaaatgaacagcctgagagccgaggacacggccgtatattactgtgtgaaagatggggcaggaggctttgactactggggccagggcaccctggtcaccgtctcgagt

SEQ ID NO: 125 - DNA, 321 bp, Artificial Sequence
  source: /note="Description of Artificial Sequence: Synthetic polynucleotide"
gacatccagttgacccagtccccatcctccctgtctgcatctgtaggagacagagtcaccatcacttgccgggcaagtcagggcattagaaatcatttaggctggtatcagcagaaaccagggaaagcccctaagcgcctaatctatgctgcatccagtttgcaaagtggggtcccatcaaggttcagcggcagtggatctgggacagaattcactctcacaatcagcagcctgcagcctgaagattttgcaacttattactgtctacagcataatagttaccctccgacgttcggccaagggaccaaggtggaaatcaag

SEQ ID NO: 126 - protein, 117 aa, Artificial Sequence
  source: /note="Description of Artificial Sequence: Synthetic polypeptide"
QVQLVESGGGLVQPGGSLRLSCTASGFTFSSYAMSWVRQAPGKGLEWVSAIGGSGGSAYYADSVKGRFTISRDNSKNTLYLQMNSLRAEDTAVYYCVKDGAGGFDYWGQGTLVTVSS

SEQ ID NO: 127 - protein, 107 aa, Artificial Sequence
  source: /note="Description of Artificial Sequence: Synthetic polypeptide"
DIQLTQSPSSLSASVGDRVTITCRASQGIRNHLGWYQQKPGKAPKRLIYAASSLQSGVPSRFSGSGSGTEFTLTISSLQPEDFATYYCLQHNSYPPTFGQGTKVEIK

SEQ ID NO: 128 - protein, 8 aa, Artificial Sequence
  source: /note="Description of Artificial Sequence: Synthetic peptide"
GFTFSSYA

SEQ ID NO: 129 - protein, 8 aa, Artificial Sequence
  source: /note="Description of Artificial Sequence: Synthetic peptide"
IGGSGGSA

SEQ ID NO: 130 - protein, 12 aa, Artificial Sequence
  source: /note="Description of Artificial Sequence: Synthetic peptide"
CVKDGAGGFDYW

SEQ ID NO: 131 - protein, 6 aa, Artificial Sequence
  source: /note="Description of Artificial Sequence: Synthetic peptide"
QGIRNH

SEQ ID NO: 132 - protein, 3 aa, Artificial Sequence
  source: /note="Description of Artificial Sequence: Synthetic peptide"
AAS

SEQ ID NO: 133 - protein, 11 aa, Artificial Sequence [sequence omitted]

SEQ ID NO: 134 - DNA, 354 bp, Artificial Sequence
  source: /note="Description of Artificial Sequence: Synthetic polynucleotide"
cagatgcagctacagcagtctgggggaggcttggtacagccgggggggtccctgagactctcctgtgcagcctctggattcaccgttagcagctatgccatgagctgggtccgccaggctctagggaaggggctggagtgggtctcaggtattagtggtagtggtggtagcacatactacgcagactccgtgaagggccggttcaccatctccagagacaattccaagaatacgctgtatctgcaaatgaacagcctgagagccgaggacacggccgtatattactgtgcgaagatagtgggagctacccactttgactactggggccagggaaccctggtcacggtctcgagt

SEQ ID NO: 135 - DNA, 339 bp, Artificial Sequence
  source: /note="Description of Artificial Sequence: Synthetic polynucleotide"
gaaattgtgatgacacagtctccagactccctggctgtgtctctgggcgagagggccaccatcaactgcaagtccagccagagtgttttatacagctccaacaataagaactacttagcttggtaccagcagaaaccaggacagcctcctaagctgctcatttactgggcatctacccgggaatccggggtccctgaccgattcagtggcagcgggtctgggacagatttcactctcaccatcagcagcctgcaggctgaagatgtggcagtttattactgtcagcaatattatagtggtccgatcaccttcggccaagggacacgactggagattaag

SEQ ID NO: 136 - protein, 118 aa, Artificial Sequence
  source: /note="Description of Artificial Sequence: Synthetic polypeptide"
QMQLQQSGGGLVQPGGSLRLSCAASGFTVSSYAMSWVRQALGKGLEWVSGISGSGGSTYYADSVKGRFTISRDNSKNTLYLQMNSLRAEDTAVYYCAKIVGATHFDYWGQGTLVTVSS

SEQ ID NO: 137 - protein, 113 aa, Artificial Sequence
  source: /note="Description of Artificial Sequence: Synthetic polypeptide"
EIVMTQSPDSLAVSLGERATINCKSSQSVLYSSNNKNYLAWYQQKPGQPPKLLIYWASTRESGVPDRFSGSGSGTDFTLTISSLQAEDVAVYYCQQYYSGPITFGQGTRLEIK

SEQ ID NO: 138 - protein, 8 aa, Artificial Sequence
  source: /note="Description of Artificial Sequence: Synthetic peptide"
GFTVSSYA

SEQ ID NO: 139 - protein, 8 aa, Artificial Sequence
  source: /note="Description of Artificial Sequence: Synthetic peptide"
ISGSGGST

SEQ ID NO: 140 - protein, 13 aa, Artificial Sequence
  source: /note="Description of Artificial Sequence: Synthetic peptide"
CAKIVGATHFDYW

SEQ ID NO: 141 - protein, 12 aa, Artificial Sequence
  source: /note="Description of Artificial Sequence: Synthetic peptide"
QSVLYSSNNKNY

SEQ ID NO: 142 - protein, 3 aa, Artificial Sequence
  source: /note="Description of Artificial Sequence: Synthetic peptide"
WAS

SEQ ID NO: 143 - protein, 11 aa, Artificial Sequence [sequence omitted]

SEQ ID NO: 144 - DNA, 366 bp, Artificial Sequence
  source: /note="Description of Artificial Sequence: Synthetic polynucleotide"
caggtgcagctggtggagtcgggcccaggactggtgaagccttcacagaccctgtccctcacctgcactgtctctggtggctccatcaacagtggtggttactactggagctggatccgccagcacccagggaagggcctggagtggattgggtacatctattacagtgggagcatctactacaacccgtccctcaggagtcgacttaccatatcagtagacacgtctaagaaccagttctccctgaagctgagctctgtgactgccgcggacacggccgtttattactgtgcgactccttattactatggttcggggagttatggggactactggggccagggcaccctggtcactgtctcgagt

SEQ ID NO: 145 - DNA, 321 bp, Artificial Sequence
  source: /note="Description of Artificial Sequence: Synthetic polynucleotide"
gacatccagatgacccagtctccagccaccctgtctttgtctccaggggaaagagccaccctctcctgcagggccagtcagagtgttaacaactacttagcctggtaccaacagaaacctggccaggctcccaggctcctcatctatgatgcatccaacagggccactggcatcccagccaggttcagtggcagtgggtctgggacagacttcactctcaccatcagcagcctagagcctgaagattttgcagtttattactgtcagcagcgtagcaactggcccatcaccttcggccaagggacacgactggagattaaa

SEQ ID NO: 146 - protein, 122 aa, Artificial Sequence
  source: /note="Description of Artificial Sequence: Synthetic polypeptide"
QVQLVESGPGLVKPSQTLSLTCTVSGGSINSGGYYWSWIRQHPGKGLEWIGYIYYSGSIYYNPSLRSRLTISVDTSKNQFSLKLSSVTAADTAVYYCATPYYYGSGSYGDYWGQGTLVTVSS

SEQ ID NO: 147 - protein, 107 aa, Artificial Sequence
  source: /note="Description of Artificial Sequence: Synthetic polypeptide"
DIQMTQSPATLSLSPGERATLSCRASQSVNNYLAWYQQKPGQAPRLLIYDASNRATGIPARFSGSGSGTDFTLTISSLEPEDFAVYYCQQRSNWPITFGQGTRLEIK

SEQ ID NO: 148 - protein, 10 aa, Artificial Sequence
  source: /note="Description of Artificial Sequence: Synthetic peptide"
GGSINSGGYY

SEQ ID NO: 149 - protein, 7 aa, Artificial Sequence
  source: /note="Description of Artificial Sequence: Synthetic peptide"
IYYSGSI

SEQ ID NO: 150 - protein, 16 aa, Artificial Sequence
  source: /note="Description of Artificial Sequence: Synthetic peptide"
CATPYYYGSGSYGDYW

SEQ ID NO: 151 - protein, 6 aa, Artificial Sequence
  source: /note="Description of Artificial Sequence: Synthetic peptide"
QSVNNY

SEQ ID NO: 152 - protein, 3 aa, Artificial Sequence
  source: /note="Description of Artificial Sequence: Synthetic peptide"
DAS

SEQ ID NO: 153 - protein, 11 aa, Artificial Sequence [sequence omitted]

SEQ ID NO: 154 - DNA, 363 bp, Artificial Sequence
  source: /note="Description of Artificial Sequence: Synthetic polynucleotide"
cagatgcagctgcaggagtcgggcccaggactggtgaagccttctcagaccctgtccctcacctgcactgtgtctggtggctccatcagcagtgttggttactactggaactggatccgccagcacccagggaagggcctggagttcattgggtacatctattacagtgggagcatctactacaatccgtccctcaagagtcgagttaccatatccgtagacacgtctaagaaccagttctccctgaagctgagctctgtgactgccgcggacacggccctatattactgtgcgagcgtcggtatagtgggagcctcctactttgagtactggggccagggaaccctggtcacagtctcgagt

SEQ ID NO: 155 - DNA, 321 bp, Artificial Sequence
  source: /note="Description of Artificial Sequence: Synthetic polynucleotide"
gaaattgtgatgacacagtctccagccaccctgtctttgtctccaggggaaagagccaccctctcctgcagggccagtcagagtgttagcagctacttagcctggtaccaacagaaacctggccaggctcccaggctcctcatctatgatgcatccaacagggccactggcatcccagccaggttcagtggcagtgggtctgggacagacttcactctcaccatcagcagcctagagcctgaagattttgcagtttattactgtcagcagcgtagcaactggcctatcaccttcggccaagggacacgactggagatcaag

SEQ ID NO: 156 - protein, 121 aa, Artificial Sequence
  source: /note="Description of Artificial Sequence: Synthetic polypeptide"
QMQLQESGPGLVKPSQTLSLTCTVSGGSISSVGYYWNWIRQHPGKGLEFIGYIYYSGSIYYNPSLKSRVTISVDTSKNQFSLKLSSVTAADTALYYCASVGIVGASYFEYWGQGTLVTVSS

SEQ ID NO: 157 - protein, 107 aa, Artificial Sequence
  source: /note="Description of Artificial Sequence: Synthetic polypeptide"
EIVMTQSPATLSLSPGERATLSCRASQSVSSYLAWYQQKPGQAPRLLIYDASNRATGIPARFSGSGSGTDFTLTISSLEPEDFAVYYCQQRSNWPITFGQGTRLEIK

SEQ ID NO: 158 - protein, 10 aa, Artificial Sequence
  source: /note="Description of Artificial Sequence: Synthetic peptide"
GGSISSVGYY

SEQ ID NO: 159 - protein, 7 aa, Artificial Sequence
  source: /note="Description of Artificial Sequence: Synthetic peptide"
IYYSGSI

SEQ ID NO: 160 - protein, 15 aa, Artificial Sequence
  source: /note="Description of Artificial Sequence: Synthetic peptide"
CASVGIVGASYFEYW

SEQ ID NO: 161 - protein, 6 aa, Artificial Sequence
  source: /note="Description of Artificial Sequence: Synthetic peptide"
QSVSSY

SEQ ID NO: 162 - protein, 3 aa, Artificial Sequence
  source: /note="Description of Artificial Sequence: Synthetic peptide"
DAS

SEQ ID NO: 163 - protein, 11 aa, Artificial Sequence [sequence omitted]

SEQ ID NO: 164 - DNA, 354 bp, Artificial Sequence
  source: /note="Description of Artificial Sequence: Synthetic polynucleotide"
caggtgcagctacagcagtctgggggaggcttggtacagcctggggggtccctgagactctcctgtgcagcctctggattcaccttaagcagctatgccatgagctgggtccgccaggctccagggaaggggctggagtgggtctcaggtattagtggtagtggtggtagcacatacaacgcagactccgtgaagggccggttcaccatctccagagacaattccaagaacacgctgtttctgcaaatgaacagcctgagagccgaggacacggccgtatattactgtgcgaaaatttttgggtcctactactttgactactggggccagggaaccctggtcacagtctcgagt

SEQ ID NO: 165 - DNA, 339 bp, Artificial Sequence
  source: /note="Description of Artificial Sequence: Synthetic polynucleotide"
gaaattgtgatgacacagtctccagactccctggctgtgtctctgggcgagagggccaccatcaactgcaagtccagccagagtgttttatacagctccaacaataagaactacttagcttggtaccagcagaaaccaggacagcctcctaagctgctcatttactggacatctacccgggaatccggggtccctaaccgattcagtggcagcgggtctgggacagatttcactctcaccatcagcagcctgcaggctgaagatgtggcagtttattactgtcagcaatattatagtggtcctccgacgttcggccaagggaccaaggtggaaatcaaa

SEQ ID NO: 166 - protein, 118 aa, Artificial Sequence
  source: /note="Description of Artificial Sequence: Synthetic polypeptide"
QVQLQQSGGGLVQPGGSLRLSCAASGFTLSSYAMSWVRQAPGKGLEWVSGISGSGGSTYNADSVKGRFTISRDNSKNTLFLQMNSLRAEDTAVYYCAKIFGSYYFDYWGQGTLVTVSS

SEQ ID NO: 167 - protein, 113 aa, Artificial Sequence
  source: /note="Description of Artificial Sequence: Synthetic polypeptide"
EIVMTQSPDSLAVSLGERATINCKSSQSVLYSSNNKNYLAWYQQKPGQPPKLLIYWTSTRESGVPNRFSGSGSGTDFTLTISSLQAEDVAVYYCQQYYSGPPTFGQGTKVEIK

SEQ ID NO: 168 - protein, 8 aa, Artificial Sequence
  source: /note="Description of Artificial Sequence: Synthetic peptide"
GFTLSSYA

SEQ ID NO: 169 - protein, 8 aa, Artificial Sequence
  source: /note="Description of Artificial Sequence: Synthetic peptide"
ISGSGGST

SEQ ID NO: 170 - protein, 13 aa, Artificial Sequence
  source: /note="Description of Artificial Sequence: Synthetic peptide"
CAKIFGSYYFDYW

SEQ ID NO: 171 - protein, 12 aa, Artificial Sequence
  source: /note="Description of Artificial Sequence: Synthetic peptide"
QSVLYSSNNKNY

SEQ ID NO: 172 - protein, 3 aa, Artificial Sequence
  source: /note="Description of Artificial Sequence: Synthetic peptide"
WTS

SEQ ID NO: 173 - protein, 11 aa, Artificial Sequence [sequence omitted]

SEQ ID NO: 174 - DNA, 354 bp, Artificial Sequence
  source: /note="Description of Artificial Sequence: Synthetic polynucleotide"
caggtgcagctggtggagtctgggggaggcttggttcggcctggggggtccctgagactctcctgtgcagtctctggattcacctttagcagctatgccatgagctgggtccgccaggctccagggaaggggctggagtgggtctcaggtattagtggtagtggtggtagcacatacaacgcagactccgtgaagggccggttcaccatctccagagacaattccaagaacacgctgtatcttcaaatgaacagcctgagagccgaggacacggccgtatattactgtgcgaaaatttttgggtcctactactttgactactggggccagggaaccctggtcaccgtctcgagt

SEQ ID NO: 175 - DNA, 339 bp, Artificial Sequence
  source: /note="Description of Artificial Sequence: Synthetic polynucleotide"
gaaattgtgatgacacagtctccagactccctggctgtgtctctgggcgagagggccaccatcaactgcaagtccagccagagtgttttatacagctccaataataagaactacttagcttggtaccagcagaaatcaggacagcctcctaagctgctcatttactgggcatctacccgggaatccggggtccctgaccgattcagtggcagcgggtctgggacagatttcactctcaccatcagcagcctgcaggctgaagatgtggcagtttattactgtcagcaatattatagtggtccaccgacgttcggccaagggaccaaggtggaaatcaaa

SEQ ID NO: 176 - protein, 118 aa, Artificial Sequence
  source: /note="Description of Artificial Sequence: Synthetic polypeptide"
QVQLVESGGGLVRPGGSLRLSCAVSGFTFSSYAMSWVRQAPGKGLEWVSGISGSGGSTYNADSVKGRFTISRDNSKNTLYLQMNSLRAEDTAVYYCAKIFGSYYFDYWGQGTLVTVSS

SEQ ID NO: 177 - protein, 113 aa, Artificial Sequence
  source: /note="Description of Artificial Sequence: Synthetic polypeptide"
EIVMTQSPDSLAVSLGERATINCKSSQSVLYSSNNKNYLAWYQQKSGQPPKLLIYWASTRESGVPDRFSGSGSGTDFTLTISSLQAEDVAVYYCQQYYSGPPTFGQGTKVEIK

SEQ ID NO: 178 - protein, 8 aa, Artificial Sequence
  source: /note="Description of Artificial Sequence: Synthetic peptide"
GFTFSSYA

SEQ ID NO: 179 - protein, 8 aa, Artificial Sequence
  source: /note="Description of Artificial Sequence: Synthetic peptide"
ISGSGGST

SEQ ID NO: 180 - protein, 13 aa, Artificial Sequence
  source: /note="Description of Artificial Sequence: Synthetic peptide"
CAKIFGSYYFDYW

SEQ ID NO: 181 - protein, 12 aa, Artificial Sequence
  source: /note="Description of Artificial Sequence: Synthetic peptide"
QSVLYSSNNKNY

SEQ ID NO: 182 - protein, 3 aa, Artificial Sequence
  source: /note="Description of Artificial Sequence: Synthetic peptide"
WAS

SEQ ID NO: 183 - protein, 11 aa, Artificial Sequence [sequence omitted]

SEQ ID NO: 184 - DNA, 377 bp, Artificial Sequence
  source: /note="Description of Artificial Sequence: Synthetic polynucleotide"
acgtgacagggcgcgcccaggtccagctgcaggagagcggtcccggactggtgaagccatcccagacactgagcctgacttgtactgtgagcggcggtagcatctccagcggcggctactattggtcctggatcaggcagcacccaggcaagggcctggagtggatcggctacatctactatagcggctctatctactataacccttccctgaagagccgggtgaccatctctgtggacacatccaagaatcagttctatctgaagctgtcttccgtgaccgccgctgatacagccgtgtactattgcgcctcactgatggtctggggggtcatgggcgattactgggggcagggcacactggtcacagtctcgagt

SEQ ID NO: 185 - DNA, 321 bp, Artificial Sequence
  source: /note="Description of Artificial Sequence: Synthetic polynucleotide"
gagattgtgctgacccagtctcccgccaccctgtctctgagtcctggcgagagagccaccctgagctgcagagcctctcagtccgtgtccagctatctggcctggtatcagcagaagcccggccaggctccccggctgctgatctacgatgcctccaatagagccaccggcatccctgccagattctccggctctggctctggcaccgactttaccctgaccatctccagcctggaacccgaggacttcgccgtgtactactgccagcagcggtccgactggcctcctacatttggccaaggcaccaaggtggaaatcaag

SEQ ID NO: 186 - protein, 120 aa, Artificial Sequence
  source: /note="Description of Artificial Sequence: Synthetic polypeptide"
QVQLQESGPGLVKPSQTLSLTCTVSGGSISSGGYYWSWIRQHPGKGLEWIGYIYYSGSIYYNPSLKSRVTISVDTSKNQFYLKLSSVTAADTAVYYCASLMVWGVMGDYWGQGTLVTVSS

SEQ ID NO: 187 - protein, 107 aa, Artificial Sequence
  source: /note="Description of Artificial Sequence: Synthetic polypeptide"
EIVLTQSPATLSLSPGERATLSCRASQSVSSYLAWYQQKPGQAPRLLIYDASNRATGIPARFSGSGSGTDFTLTISSLEPEDFAVYYCQQRSDWPPTFGQGTKVEIK

SEQ ID NO: 188 - protein, 10 aa, Artificial Sequence
  source: /note="Description of Artificial Sequence: Synthetic peptide"
GGSISSGGYY

SEQ ID NO: 189 - protein, 7 aa, Artificial Sequence
  source: /note="Description of Artificial Sequence: Synthetic peptide"
IYYSGSI

SEQ ID NO: 190 - protein, 14 aa, Artificial Sequence
  source: /note="Description of Artificial Sequence: Synthetic peptide"
CASLMVWGVMGDYW

SEQ ID NO: 191 - protein, 6 aa, Artificial Sequence
  source: /note="Description of Artificial Sequence: Synthetic peptide"
QSVSSY

SEQ ID NO: 192 - protein, 3 aa, Artificial Sequence
  source: /note="Description of Artificial Sequence: Synthetic peptide"
DAS

SEQ ID NO: 193 - protein, 11 aa, Artificial Sequence [sequence omitted]

SEQ ID NO: 194 - DNA, 354 bp, Artificial Sequence
  source: /note="Description of Artificial Sequence: Synthetic polynucleotide"
caggtccagctacagcagtctgggggaggcttggttcatcctggggggtccctaagactctcctgtgcagcctctggattcaccgttgacacctatgccatgacctgggtccgccaggctccagggaaggggctggagtgggtctcaggtattagcggtagtggtggtagcacatactacgcagactccgtgaagggccggttcaccatctccagagacaactccaagaacacgctgtatctgcaaatgaacagcctgagagacgaggacacggccgtatattactgtgcgaagatagtgggagttacccactttgactactggggccagggcaccctggtcacggtctcgagt

SEQ ID NO: 195 - DNA, 339 bp, Artificial Sequence
  source: /note="Description of Artificial Sequence: Synthetic polynucleotide"
gaaattgtgatgacgcagtctccagactccctggctgtgtctctgggcgagagggccaccatcaactgcaagtccagccagagtgttttatacaggtccaacaataagaactatttagcttggtaccagcagaaaccaggacagcctcctaagctgctcatttactgggcatctacccgggaatccggggtccctgaccgattcagtggcagcgggtctgggacagatttcactctcaccatcagcagcctgcaggctgaagatgtggcagtttattactgtcagcaatattatagtggtccgatcaccttcggccaagggacacgactggagattaag

SEQ ID NO: 196 - protein, 118 aa, Artificial Sequence
  source: /note="Description of Artificial Sequence: Synthetic polypeptide"
QVQLQQSGGGLVHPGGSLRLSCAASGFTVDTYAMTWVRQAPGKGLEWVSGISGSGGSTYYADSVKGRFTISRDNSKNTLYLQMNSLRDEDTAVYYCAKIVGVTHFDYWGQGTLVTVSS

SEQ ID NO: 197 - protein, 113 aa, Artificial Sequence
  source: /note="Description of Artificial Sequence: Synthetic polypeptide"
EIVMTQSPDSLAVSLGERATINCKSSQSVLYRSNNKNYLAWYQQKPGQPPKLLIYWASTRESGVPDRFSGSGSGTDFTLTISSLQAEDVAVYYCQQYYSGPITFGQGTRLEIK

SEQ ID NO: 198 - protein, 8 aa, Artificial Sequence
  source: /note="Description of Artificial Sequence: Synthetic peptide"
GFTVDTYA

SEQ ID NO: 199 - protein, 8 aa, Artificial Sequence
  source: /note="Description of Artificial Sequence: Synthetic peptide"
ISGSGGST

SEQ ID NO: 200 - protein, 13 aa, Artificial Sequence
  source: /note="Description of Artificial Sequence: Synthetic peptide"
CAKIVGVTHFDYW

SEQ ID NO: 201 - protein, 12 aa, Artificial Sequence
  source: /note="Description of Artificial Sequence: Synthetic peptide"
QSVLYRSNNKNY

SEQ ID NO: 202 - protein, 3 aa, Artificial Sequence
  source: /note="Description of Artificial Sequence: Synthetic peptide"
WAS

SEQ ID NO: 203 - protein, 11 aa, Artificial Sequence [sequence omitted]

SEQ ID NO: 204 - DNA, 369 bp, Artificial Sequence
  source: /note="Description of Artificial Sequence: Synthetic polynucleotide"
caggtcaccttgaaggagtcgggcccaggactggtgaagccttcacagaccctgtccctcacctgcactgtctctggtggctccatcagcagtggtggtcattactggagctggatccgccagcacccagggaagggcctggagtggattgggtacatctcttacagtgggagcacctactacaacccgtccctcaagagtcgacttaccatatcagtagacacgtctaagaaccagttctccctgaagctgagctctgtgactgccgcggacacggccgtgtattactgtgcgaccgcgtattacgatattttgactggttacccttttgactactggggccagggaaccctggtcacggtctcgagt

SEQ ID NO: 205 - DNA, 321 bp, Artificial Sequence
  source: /note="Description of Artificial Sequence: Synthetic polynucleotide"
gaaattgtgatgacacagtctccagccaccctgtctttgtctccaggggaaagagccaccctctcctgcagggccagtcagagtgttagcagctacttagcctggtaccaacagaaacctggccaggctcccaggctcctcatctatgatgcatccgacagggccactggcatcccagccaggttcagtggcagtgggtctgggacagacttcactctcaccatcagcagcctagagcctgaagattttgcagtttattactgtcagcagcgtagcaactggccgatcaccttcggccaagggacacgactggagatcaag

SEQ ID NO: 206 - protein, 123 aa, Artificial Sequence
  source: /note="Description of Artificial Sequence: Synthetic polypeptide"
QVTLKESGPGLVKPSQTLSLTCTVSGGSISSGGHYWSWIRQHPGKGLEWIGYISYSGSTYYNPSLKSRLTISVDTSKNQFSLKLSSVTAADTAVYYCATAYYDILTGYPFDYWGQGTLVTVSS

SEQ ID NO: 207 - protein, 107 aa, Artificial Sequence
  source: /note="Description of Artificial Sequence: Synthetic polypeptide"
EIVMTQSPATLSLSPGERATLSCRASQSVSSYLAWYQQKPGQAPRLLIYDASDRATGIPARFSGSGSGTDFTLTISSLEPEDFAVYYCQQRSNWPITFGQGTRLEIK

SEQ ID NO: 208 - protein, 10 aa, Artificial Sequence
  source: /note="Description of Artificial Sequence: Synthetic peptide"
GGSISSGGHY

SEQ ID NO: 209 - protein, 7 aa, Artificial Sequence
  source: /note="Description of Artificial Sequence: Synthetic peptide"
ISYSGST

SEQ ID NO: 210 - protein, 17 aa, Artificial Sequence
  source: /note="Description of Artificial Sequence: Synthetic peptide"
CATAYYDILTGYPFDYW

SEQ ID NO: 211 - protein, 6 aa, Artificial Sequence
  source: /note="Description of Artificial Sequence: Synthetic peptide"
QSVSSY

SEQ ID NO: 212 - protein, 3 aa, Artificial Sequence
  source: /note="Description of Artificial Sequence: Synthetic peptide"
DAS

SEQ ID NO: 213 - protein, 11 aa, Artificial Sequence [sequence omitted]

SEQ ID NO: 214 - DNA, 369 bp, Artificial Sequence
  source: /note="Description of Artificial Sequence: Synthetic polynucleotide"
caggtgcagctacagcagtcgggcccaggactggtgaagccttcacagaccctgtccctcacctgcactgtctctggtggctccatcagcagtggtggttactactggagctggatccgccagcacccagggaagggcctggagtggattgggtacatctcttatagtgggagtatctactacaacccgtccctcaagagtcgagttaccatatcagtagacacgtctaagaaccagttctccctgaagctgagctctgtgactgccacggacacggccgtgtattactgtgcgaccgcgtattacgatcttttgactggttacccttttgactactggggccagggaaccctggtcacggtctcgagt

SEQ ID NO: 215 - DNA, 321 bp, Artificial Sequence
  source: /note="Description of Artificial Sequence: Synthetic polynucleotide"
gaaattgtgatgacgcagtctccagccaccctgtctttgtctccaggggaaagagccaccctctcctgcagggccagtcagagtgttagcagctacttagcctggtaccaacagaaacctggccaggctcccaggctcctcatctatgatgcatccaacagggccactggcatcccagccaggttcagtggcagtgggtctgggacagacttcactctcaccatcagcagcctagagcctgaagattttgcagtttattactgtcagcagcgtagcaactggccgatcaccttcggccaagggacacgactggagattaag

SEQ ID NO: 216 - protein, 123 aa, Artificial Sequence
  source: /note="Description of Artificial Sequence: Synthetic polypeptide"
QVQLQQSGPGLVKPSQTLSLTCTVSGGSISSGGYYWSWIRQHPGKGLEWIGYISYSGSIYYNPSLKSRVTISVDTSKNQFSLKLSSVTATDTAVYYCATAYYDLLTGYPFDYWGQGTLVTVSS

SEQ ID NO: 217 - protein, 107 aa, Artificial Sequence; identical to SEQ ID NO: 157
  source: /note="Description of Artificial Sequence: Synthetic polypeptide"

SEQ ID NO: 218 - protein, 10 aa, Artificial Sequence
  source: /note="Description of Artificial Sequence: Synthetic peptide"
GGSISSGGYY

SEQ ID NO: 219 - protein, 7 aa, Artificial Sequence
  source: /note="Description of Artificial Sequence: Synthetic peptide"
ISYSGSI

SEQ ID NO: 220 - protein, 17 aa, Artificial Sequence
  source: /note="Description of Artificial Sequence: Synthetic peptide"
CATAYYDLLTGYPFDYW

SEQ ID NO: 221 - protein, 6 aa, Artificial Sequence
  source: /note="Description of Artificial Sequence: Synthetic peptide"
QSVSSY

SEQ ID NO: 222 - protein, 3 aa, Artificial Sequence
  source: /note="Description of Artificial Sequence: Synthetic peptide"
DAS

SEQ ID NO: 223 - protein, 11 aa, Artificial Sequence [sequence omitted]

SEQ ID NO: 224 - DNA, 379 bp, Artificial Sequence
  source: /note="Description of Artificial Sequence: Synthetic polynucleotide"
ggcgcgccgaggtgcagctgctggaatctggaggaggactggtccagccaggtggatccctgcgactgagctgcgccgcttctggattcacctttacaagatacgacatggtgtgggtccgccaggcaccaggaaagggactggagtgggtggctggtatcggcgatagtaacaagatgacccgctacgcacctgccgtcaaagggagggcaacaattagtcgggacaactcaaagaatactctgtatctgcagatgaattccctgcgagctgaggatacagcagtgtactattgtgccaaaggtagctgcatcgcctgttgggacgaagctggccgtattgatgcatggggacaggggactctggtgaccgtctcgag

SEQ ID NO: 225 - DNA, 351 bp, Artificial Sequence
  source: /note="Description of Artificial Sequence: Synthetic polynucleotide"
gctagcctcttacgagctgactcaggaccctgcagtgagtgtcgccctgggccagacagtgagaatcacttgctccggcggagggagctacgatggttccagctactatggctggtatcagcagaagccaggacaggcacctgtgaccgtcatctataacaataacaataggccatctgacattcccgatcggttcagtggatctagttcagggaacacagcttctctgaccattacaggagcccaggctgaggacgaagcagattactattgtgggtcatacgacaggccagaaacaaattccgattatgtgggaatgtttggtagcggcactaaagtcaccgtcctagg

SEQ ID NO: 226 - protein, 124 aa, Artificial Sequence
  source: /note="Description of Artificial Sequence: Synthetic polypeptide"
EVQLLESGGGLVQPGGSLRLSCAASGFTFTRYDMVWVRQAPGKGLEWVAGIGDSNKMTRYAPAVKGRATISRDNSKNTLYLQMNSLRAEDTAVYYCAKGSCIACWDEAGRIDAWGQGTLVTVSS

SEQ ID NO: 227 - protein, 114 aa, Artificial Sequence
  source: /note="Description of Artificial Sequence: Synthetic polypeptide"
SYELTQDPAVSVALGQTVRITCSGGGSYDGSSYYGWYQQKPGQAPVTVIYNNNNRPSDIPDRFSGSSSGNTASLTITGAQAEDEADYYCGSYDRPETNSDYVGMFGSGTKVTVL

SEQ ID NO: 228 - protein, 8 aa, Artificial Sequence
  source: /note="Description of Artificial Sequence: Synthetic peptide"
GFTFTRYD

SEQ ID NO: 229 - protein, 8 aa, Artificial Sequence
  source: /note="Description of Artificial Sequence: Synthetic peptide"
IGDSNKMT

SEQ ID NO: 230 - protein, 19 aa, Artificial Sequence
  source: /note="Description of Artificial Sequence: Synthetic peptide"
CAKGSCIACWDEAGRIDAW

SEQ ID NO: 231 - protein, 8 aa, Artificial Sequence
  source: /note="Description of Artificial Sequence: Synthetic peptide"
GSYDGSSY

SEQ ID NO: 232 - protein, 3 aa, Artificial Sequence
  source: /note="Description of Artificial Sequence: Synthetic peptide"
NNN

SEQ ID NO: 233 - protein, 17 aa, Artificial Sequence
  source: /note="Description of Artificial Sequence: Synthetic peptide"
CGSYDRPETNSDYVGMF

SEQ ID NO: 234 - DNA, 400 bp, Artificial Sequence
  source: /note="Description of Artificial Sequence: Synthetic polynucleotide"
ggcgcgccgaggtgcagctgctggaaagcggaggaggactggtccagccaggtggatctctgcgactgagttgcgccgcttcaggcttcacattttctgactacgccatgaactgggtgaggcaggctcctggcaagggactggagtgggtcgcaggaatcgggaacgatggaagttacactaattatggagcagccgtgaaggggagagctactatttcccgcgacaacagcaaaaataccctgtacctgcagatgaactcactgagagctgaagataccgcagtgtactattgtgcctctgacatcaggagtcggaatgattgctcctatttcctgggagggtgttccagcggctttattgacgtgtggggtcagggcaccctggtcacagtctcgag

SEQ ID NO: 235 - DNA, 321 bp, Artificial Sequence
  source: /note="Description of Artificial Sequence: Synthetic polynucleotide"
gctagcctcttacgagctgacccaggacccagcagtgtccgtcgccctgggccagacagtgagaatcacttgctccggcggatccagctacagctatgggtggttccagcagaagcccggtcaggcccctgtgaccgtcatctatgaaagtaacaataggccatcagacattcccgatcggttttctggctctagttcaggaaacacagctagtctgaccatcacaggggcccaggctgaggacgaagctgattactattgtggcaatgcagattccagctctggaattttcgggtccggtactaaagtcaccgtcctagg

SEQ ID NO: 236 - protein, 131 aa, Artificial Sequence
  source: /note="Description of Artificial Sequence: Synthetic polypeptide"
EVQLLESGGGLVQPGGSLRLSCAASGFTFSDYAMNWVRQAPGKGLEWVAGIGNDGSYTNYGAAVKGRATISRDNSKNTLYLQMNSLRAEDTAVYYCASDIRSRNDCSYFLGGCSSGFIDVWGQGTLVTVSS

SEQ ID NO: 237 - protein, 104 aa, Artificial Sequence
  source: /note="Description of Artificial Sequence: Synthetic polypeptide"
SYELTQDPAVSVALGQTVRITCSGGSSYSYGWFQQKPGQAPVTVIYESNNRPSDIPDRFSGSSSGNTASLTITGAQAEDEADYYCGNADSSSGIFGSGTKVTVL

SEQ ID NO: 238 - protein, 8 aa, Artificial Sequence
  source: /note="Description of Artificial Sequence: Synthetic peptide"
GFTFSDYA

SEQ ID NO: 239 - protein, 8 aa, Artificial Sequence
  source: /note="Description of Artificial Sequence: Synthetic peptide"
IGNDGSYT

SEQ ID NO: 240 - protein, 26 aa, Artificial Sequence
  source: /note="Description of Artificial Sequence: Synthetic peptide"
CASDIRSRNDCSYFLGGCSSGFIDVW

SEQ ID NO: 241 - protein, 4 aa, Artificial Sequence
  source: /note="Description of Artificial Sequence: Synthetic peptide"
SSYS

SEQ ID NO: 242 - protein, 3 aa, Artificial Sequence
  source: /note="Description of Artificial Sequence: Synthetic peptide"
ESN

SEQ ID NO: 243 - protein, 11 aa, Artificial Sequence
  source: /note="Description of Artificial Sequence: Synthetic peptide"
CGNADSSSGIF

SEQ ID NO: 244 - DNA, 385 bp, Artificial Sequence
  source: /note="Description of Artificial Sequence: Synthetic polynucleotide"
ggcgcgccgaggtgcagctgctggaatccggaggaggactggtccagccaggtggatccctgcgactgagctgcgccgcttctggattcgactttagcgatcacgggatgcagtgggtgagacaggcaccaggcaagggactggagtacgtgggtgtcatcgacaccacaggccgctatacatactatgcacctgccgtcaagggcagggctaccattagtcgggacaactcaaaaaatacactgtacctgcagatgaactctctgagggctgaagatactgcagtgtactattgcgccaaaactacctgcgtgggagggtacctgtgcaataccgtcggaagtatcgatgcttggggacaggggacactggtgactgtctcgag

SEQ ID NO: 245 - DNA, 330 bp, Artificial Sequence
  source: /note="Description of Artificial Sequence: Synthetic polynucleotide"
gctagcctcctacgagctgactcaggacccagcagtgagcgtcgccctgggccagacagtgagaatcacttgctctggcggagggtccagctcttactatggttggtaccagcagaagcccggccaggctcctgtgaccgtcatctatgacgatacaaacaggccaagtggaattcccgatcggttctcaggtagttcatccggcaatacagcttctctgaccatcacaggggcccaggctgaggacgaagcagattactattgtggtggctatgaaggaagctctcacgccgggatttttggaagtgggactaaagtcaccgtcctagg

SEQ ID NO: 246 - protein, 126 aa, Artificial Sequence
  source: /note="Description of Artificial Sequence: Synthetic polypeptide"
EVQLLESGGGLVQPGGSLRLSCAASGFDFSDHGMQWVRQAPGKGLEYVGVIDTTGRYTYYAPAVKGRATISRDNSKNTLYLQMNSLRAEDTAVYYCAKTTCVGGYLCNTVGSIDAWGQGTLVTVSS

SEQ ID NO: 247 - protein, 107 aa, Artificial Sequence
  source: /note="Description of Artificial Sequence: Synthetic polypeptide"
SYELTQDPAVSVALGQTVRITCSGGGSSSYYGWYQQKPGQAPVTVIYDDTNRPSGIPDRFSGSSSGNTASLTITGAQAEDEADYYCGGYEGSSHAGIFGSGTKVTVL

SEQ ID NO: 248 - protein, 8 aa, Artificial Sequence
  source: /note="Description of Artificial Sequence: Synthetic peptide"
GFDFSDHG

SEQ ID NO: 249 - protein, 8 aa, Artificial Sequence
  source: /note="Description of Artificial Sequence: Synthetic peptide"
IDTTGRYT

SEQ ID NO: 250 - protein, 21 aa, Artificial Sequence
  source: /note="Description of Artificial Sequence: Synthetic peptide"
CAKTTCVGGYLCNTVGSIDAW

SEQ ID NO: 251 - protein, 5 aa, Artificial Sequence
  source: /note="Description of Artificial Sequence: Synthetic peptide"
GSSSY

SEQ ID NO: 252 - protein, 3 aa, Artificial Sequence
  source: /note="Description of Artificial Sequence: Synthetic peptide"
DDT

SEQ ID NO: 253 - protein, 13 aa, Artificial Sequence
  source: /note="Description of Artificial Sequence: Synthetic peptide"
CGGYEGSSHAGIF

SEQ ID NO: 254 - DNA, 376 bp, Artificial Sequence
  source: /note="Description of Artificial Sequence: Synthetic polynucleotide"
ggcgcgccgaggtgcagctgctggaaagtggaggaggactggtccagccaggtggaagcctgagactgtcttgcgccgctagtggcttcgacttttccagctacaccatgcagtgggtgaggcaggcaccaggcaagggactggagtgggtgggcgtcatctctagtactggagggtctaccggatacgggcctgctgtgaagggaagggcaacaatttcacgggataactccaaaaatactctgtatctgcagatgaacagcctgagggcagaagacacagccgtgtactattgcgtgaaatcaatctccggagatgcctggtctgtggacgggctggatgcttggggtcagggcaccctggtcacagtctcgag

SEQ ID NO: 255 - DNA, 321 bp, Artificial Sequence
  source: /note="Description of Artificial Sequence: Synthetic polynucleotide"
gctagcctcatacgagctgacccaggacccagcagtgtccgtcgccctgggacagacagtgagaatcacttgctccggaggaggatccgcctacggttggtatcagcagaagcccggccaggcacctgtgaccgtcatctactataacaatcagaggccatctggcattcccgaccggttcagtggatccagctctgggaacacagcaagtctgaccatcacaggcgcccaggctgaggacgaagccgattactattgtggaagctatgatagttcagctgtggggatttttggttctggcactaaagtcaccgtcctagg

SEQ ID NO: 256 - protein, 123 aa, Artificial Sequence
  source: /note="Description of Artificial Sequence: Synthetic polypeptide"
EVQLLESGGGLVQPGGSLRLSCAASGFDFSSYTMQWVRQAPGKGLEWVGVISSTGGSTGYGPAVKGRATISRDNSKNTLYLQMNSLRAEDTAVYYCVKSISGDAWSVDGLDAWGQGTLVTVSS

SEQ ID NO: 257 - protein, 104 aa, Artificial Sequence
  source: /note="Description of Artificial Sequence: Synthetic polypeptide"
SYELTQDPAVSVALGQTVRITCSGGGSAYGWYQQKPGQAPVTVIYYNNQRPSGIPDRFSGSSSGNTASLTITGAQAEDEADYYCGSYDSSAVGIFGSGTKVTVL

SEQ ID NO: 258 - protein, 8 aa, Artificial Sequence
  source: /note="Description of Artificial Sequence: Synthetic peptide"
GFDFSSYT

SEQ ID NO: 259 - protein, 8 aa, Artificial Sequence
  source: /note="Description of Artificial Sequence: Synthetic peptide"
ISSTGGST

SEQ ID NO: 260 - protein, 18 aa, Artificial Sequence
  source: /note="Description of Artificial Sequence: Synthetic peptide"
CVKSISGDAWSVDGLDAW

SEQ ID NO: 261 - protein, 3 aa, Artificial Sequence
  source: /note="Description of Artificial Sequence: Synthetic peptide"
GSA

SEQ ID NO: 262 - protein, 3 aa, Artificial Sequence
  source: /note="Description of Artificial Sequence: Synthetic peptide"
YNN

SEQ ID NO: 263 - protein, 12 aa, Artificial Sequence
  source: /note="Description of Artificial Sequence: Synthetic peptide"
CGSYDSSAVGIF

SEQ ID NO: 264 - DNA, 376 bp, Artificial Sequence
  source: /note="Description of Artificial Sequence: Synthetic polynucleotide"
ggcgcgccgaggtgcagctgctggaaagtggaggaggactggtccagccaggtggaagcctgagactgtcttgcgccgctagtggcttcgacttttccagctacaccatgcagtgggtgaggcaggcaccaggcaagggactggagtgggtgggcgtcatctctagtactggagggtctaccggatacgggcctgctgtgaagggaagggcaacaatttcacgggataactccaaaaatactctgtatctgcagatgaacagcctgagggcagaagacacagccgtgtactattgcgtgaaatcagtctccggagatgcctggtctgtggacgggctggatgcttggggtcagggcaccctggtcacagtctcgag

SEQ ID NO: 265 - DNA, 321 bp, Artificial Sequence
  source: /note="Description of Artificial Sequence: Synthetic polynucleotide"
gctagcctcatacgagctgacccaggacccagcagtgtccgtcgccctgggccagacagtgagaatcacttgctccggaggaggatccgcctacggttggtatcagcagaagcccggccaggcacctgtgaccgtcatctactataacaatcagaggccatctgacattcccgatcggttcagtggatccagctctgggaacacagcaagtctgaccatcacaggcgcccaggctgaggacgaagccgattactattgtggaagctatgatagttcagctgtggggatttttggttctggcactaaagtcaccgtcctagg

SEQ ID NO: 266 - protein, 123 aa, Artificial Sequence
  source: /note="Description of Artificial Sequence: Synthetic polypeptide"
EVQLLESGGGLVQPGGSLRLSCAASGFDFSSYTMQWVRQAPGKGLEWVGVISSTGGSTGYGPAVKGRATISRDNSKNTLYLQMNSLRAEDTAVYYCVKSVSGDAWSVDGLDAWGQGTLVTVSS

SEQ ID NO: 267 - protein, 104 aa, Artificial Sequence
  source: /note="Description of Artificial Sequence: Synthetic polypeptide"
SYELTQDPAVSVALGQTVRITCSGGGSAYGWYQQKPGQAPVTVIYYNNQRPSDIPDRFSGSSSGNTASLTITGAQAEDEADYYCGSYDSSAVGIFGSGTKVTVL

SEQ ID NO: 268 - protein, 8 aa, Artificial Sequence
  source: /note="Description of Artificial Sequence: Synthetic peptide"
GFDFSSYT

SEQ ID NO: 269 - protein, 8 aa, Artificial Sequence
  source: /note="Description of Artificial Sequence: Synthetic peptide"
ISSTGGST

SEQ ID NO: 270 - protein, 18 aa, Artificial Sequence
  source: /note="Description of Artificial Sequence: Synthetic peptide"
CVKSVSGDAWSVDGLDAW

SEQ ID NO: 271 - protein, 3 aa, Artificial Sequence
  source: /note="Description of Artificial Sequence: Synthetic peptide"
GSA

SEQ ID NO: 272 - protein, 3 aa, Artificial Sequence
  source: /note="Description of Artificial Sequence: Synthetic peptide"
YNN

SEQ ID NO: 273 - protein, 12 aa, Artificial Sequence
  source: /note="Description of Artificial Sequence: Synthetic peptide"
CGSYDSSAVGIF

SEQ ID NO: 274 - DNA, 385 bp, Artificial Sequence
  source: /note="Description of Artificial Sequence: Synthetic polynucleotide"
ggcgcgccgaggtgcagctgctggaatccggaggaggactggtccagccaggtggaagcctgcgactgtcttgcgccgctagtggattcgacttttccagctacggaatgcagtgggtgaggcaggcaccaggcaagggactggagtgggtgggcgtcatctctggaagtgggattaccacactgtacgcacctgccgtcaagggaagggctactatctcacgggacaactctaaaaatacagtgtatctgcagatgaactccctgagagctgaagataccgcagtctactattgtacacgctcaccctccatcacagacggctggacttatggaggggcctggattgatgcttggggtcagggcactctggtgaccgtctcgag

SEQ ID NO: 275 - DNA, 318 bp, Artificial Sequence
  source: /note="Description of Artificial Sequence: Synthetic polynucleotide"
gctagccagctacgagctgacccaggacccagcagtgtccgtcgccctgggccagacagtgagaatcacttgcagtggcggagatgggtcatacggttggttccagcagaagcccggacaggcccctgtgaccgtcatctatgacaacgataataggccatctgacattcccgatcggtttagtggctccagctctggaaacacagcttctctgaccatcacaggggcccaggctgaggacgaagctgattactattgtggcaatgcagacctgtccgggggtattttcggcagcggaactaaagtcaccgtcctagg

SEQ ID NO: 276 - protein, 126 aa, Artificial Sequence
  source: /note="Description of Artificial Sequence: Synthetic polypeptide"
EVQLLESGGGLVQPGGSLRLSCAASGFDFSSYGMQWVRQAPGKGLEWVGVISGSGITTLYAPAVKGRATISRDNSKNTVYLQMNSLRAEDTAVYYCTRSPSITDGWTYGGAWIDAWGQGTLVTVSS

SEQ ID NO: 277 - protein, 103 aa, Artificial Sequence
  source: /note="Description of Artificial Sequence: Synthetic polypeptide"
SYELTQDPAVSVALGQTVRITCSGGDGSYGWFQQKPGQAPVTVIYDNDNRPSDIPDRFSGSSSGNTASLTITGAQAEDEADYYCGNADLSGGIFGSGTKVTVL

SEQ ID NO: 278 - protein, 8 aa, Artificial Sequence
  source: /note="Description of Artificial Sequence: Synthetic peptide"
GFDFSSYG

SEQ ID NO: 279 - protein, 8 aa, Artificial Sequence
  source: /note="Description of Artificial Sequence: Synthetic peptide"
ISGSGITT

SEQ ID NO: 280 - protein, 21 aa, Artificial Sequence
  source: /note="Description of Artificial Sequence: Synthetic peptide"
CTRSPSITDGWTYGGAWIDAW

SEQ ID NO: 281 - protein, 3 aa, Artificial Sequence
  source: /note="Description of Artificial Sequence: Synthetic peptide"
DGS

SEQ ID NO: 282 - protein, 3 aa, Artificial Sequence
  source: /note="Description of Artificial Sequence: Synthetic peptide"
DND

SEQ ID NO: 283 - protein, 11 aa, Artificial Sequence
  source: /note="Description of Artificial Sequence: Synthetic peptide"
CGNADLSGGIF

SEQ ID NO: 284 - DNA, 388 bp, Artificial Sequence
  source: /note="Description of Artificial Sequence: Synthetic polynucleotide"
ggcgcgccgaggtgcagctgctggaatctggaggaggactggtccagccaggtggatccctgagactgagctgcgccgcttctggattcacctttagtacattcaacatggtgtgggtcaggcaggcacctggaaagggactggagtacgtggctgaaatctccagcgacggctcttttacatggtatgcaactgccgtcaagggcagggccaccattagtcgggataactcaaaaaatacagtgtacctgcagatgaattccctgagggctgaggacaccgcagtctactattgcgcaaaatccgattgttctagttcatactatggatatagctgtatcgggatcattgacgcttggggtcagggcactctggtgaccgtctcgag

SEQ ID NO: 285 - DNA, 339 bp, Artificial Sequence
  source: /note="Description of Artificial Sequence: Synthetic polynucleotide"
gctagcctcctatgagctgacccaggacccagcagtgagcgtcgccctgggccagacagtgagaatcacttgctccggcggaattagcgacgatggctcttactattacggatggttccagcagaagcccggacaggcccctgtgaccgtcatctatattaacgacaggcggccaagtaatatccccgataggttttcagggtccagctctggtaacacagcttctctgaccattacaggggcccaggctgaggacgaagctgattattactgtggctcttacgatagttcagcaggggtgggtatcttcggcagtggaactaaagtcaccgtcctagg

SEQ ID NO: 286 - protein, 127 aa, Artificial Sequence
  source: /note="Description of Artificial Sequence: Synthetic polypeptide"
EVQLLESGGGLVQPGGSLRLSCAASGFTFSTFNMVWVRQAPGKGLEYVAEISSDGSFTWYATAVKGRATISRDNSKNTVYLQMNSLRAEDTAVYYCAKSDCSSSYYGYSCIGIIDAWGQGTLVTVSS

SEQ ID NO: 287 - protein, 110 aa, Artificial Sequence
  source: /note="Description of Artificial Sequence: Synthetic polypeptide"
SYELTQDPAVSVALGQTVRITCSGGISDDGSYYYGWFQQKPGQAPVTVIYINDRRPSNIPDRFSGSSSGNTASLTITGAQAEDEADYYCGSYDSSAGVGIFGSGTKVTVL

SEQ ID NO: 288 - protein, 8 aa, Artificial Sequence
  source: /note="Description of Artificial Sequence: Synthetic peptide"
GFTFSTFN

SEQ ID NO: 289 - protein, 8 aa, Artificial Sequence
  source: /note="Description of Artificial Sequence: Synthetic peptide"
ISSDGSFT

SEQ ID NO: 290 - protein, 22 aa, Artificial Sequence
  source: /note="Description of Artificial Sequence: Synthetic peptide"
CAKSDCSSSYYGYSCIGIIDAW

SEQ ID NO: 291 - protein, 8 aa, Artificial Sequence
  source: /note="Description of Artificial Sequence: Synthetic peptide"
ISDDGSYY

SEQ ID NO: 292 - protein, 3 aa, Artificial Sequence
  source: /note="Description of Artificial Sequence: Synthetic peptide"
IND

SEQ ID NO: 293 - protein, 13 aa, Artificial Sequence
  source: /note="Description of Artificial Sequence: Synthetic peptide"
CGSYDSSAGVGIF

SEQ ID NO: 294 - DNA, 400 bp, Artificial Sequence
  source: /note="Description of Artificial Sequence: Synthetic polynucleotide"
ggcgcgccgaggtgcagctgctggaaagtggaggaggactggtccagccaggtggatcactgagactgtcctgcgccgcctccggcttcaccttttccagctacaacatgttctgggtgcgccaggcaccaggaaagggactggagtttgtcgctgaaatctctggtagtaatactggaagccgaacctggtacgcacctgccgtgaagggcagggctacaatttctcgggacaacagtaaaaatactctgtatctgcagatgaactctctgagggctgaggatacagcagtgtactattgtgcaaaatcaatctacggagggtattgcgccggtggctattcctgtggtgtgggcctgattgacgcatggggacaggggaccctggtcacagtctcgag

SEQ ID NO: 295 - DNA, 321 bp, Artificial Sequence
  source: /note="Description of Artificial Sequence: Synthetic polynucleotide"
gctagcctcatacgagctgacccaggacccagcagtgtccgtcgccctgggccagacagtgagaatcacttgcagtggcggatccagcgattactatgggtggttccagcagaagcccggtcaggcccctgtgaccgtcatctactataacaacaagaggccatctgacattcccgatcggtttagtggctctagttcaggaaacacagcctccctgaccattacaggggcccaggctgaggacgaagctgattactattgtggcaatgcagactccagcgtgggagtcttcgggtctggtactaaggtgaccgtcctagg

SEQ ID NO: 296 - protein, 131 aa, Artificial Sequence
  source: /note="Description of Artificial Sequence: Synthetic polypeptide"
EVQLLESGGGLVQPGGSLRLSCAASGFTFSSYNMFWVRQAPGKGLEFVAEISGSNTGSRTWYAPAVKGRATISRDNSKNTLYLQMNSLRAEDTAVYYCAKSIYGGYCAGGYSCGVGLIDAWGQGTLVTVSS

SEQ ID NO: 297 - protein, 104 aa, Artificial Sequence
  source: /note="Description of Artificial Sequence: Synthetic polypeptide"
SYELTQDPAVSVALGQTVRITCSGGSSDYYGWFQQKPGQAPVTVIYYNNKRPSDIPDRFSGSSSGNTASLTITGAQAEDEADYYCGNADSSVGVFGSGTKVTVL

SEQ ID NO: 298 - protein, 8 aa, Artificial Sequence
  source: /note="Description of Artificial Sequence: Synthetic peptide"
GFTFSSYN

SEQ ID NO: 299 - protein, 10 aa, Artificial Sequence
  source: /note="Description of Artificial Sequence: Synthetic peptide"
ISGSNTGSRT

SEQ ID NO: 300 - protein, 24 aa, Artificial Sequence
  source: /note="Description of Artificial Sequence: Synthetic peptide"
CAKSIYGGYCAGGYSCGVGLIDAW

SEQ ID NO: 301 - protein, 4 aa, Artificial Sequence
  source: /note="Description of Artificial Sequence: Synthetic peptide"
SSDY

SEQ ID NO: 302 - protein, 3 aa, Artificial Sequence
  source: /note="Description of Artificial Sequence: Synthetic peptide"
YNN

SEQ ID NO: 303 - protein, 11 aa, Artificial Sequence
  source: /note="Description of Artificial Sequence: Synthetic peptide"
CGNADSSVGVF

SEQ ID NO: 304 - DNA, 357 bp, Artificial Sequence
  source: /note="Description of Artificial Sequence: Synthetic polynucleotide"
caggtgcagctgcagcagtggggtgccggtctgctgaagccttctgaaactctgtctctgacttgtgccgtctatggtggatcattcagcggctactattggtcctggatcaggcagccccctggcaagggcctggagtggatcggcgagatcaaccaccggggctctaccaactacaatccctctctgaagagcagggtgaccatctccgtggacacatctaagaatcagttcagcctgaagctgagctccgtgaccgccgctgatacagccgtgtactattgcacaaggggggaggaatgggagtcactgttctttgattactgggggcaggggacactggtcacagtctcgagt

SEQ ID NO: 305 - DNA, 321 bp, Artificial Sequence
  source: /note="Description of Artificial Sequence: Synthetic polynucleotide"
gaaatcgtcctgacccagtcccccgccaccctgagcctgagccccggagaaagagccaccctgtcctgccgagcaagccagtccatcagctcctatctcgcctggtatcagcagaaaccaggccaggctccccggctgctgatctacggcgcctccaacagagctacaggaatcccagcccgcttcagcggctccggctctggcacagactttaccctgacaatctctagcctggagcctgaggatttcgccgtgtactattgccagcagagatctaattggccactgacattcggcggcggcacacgggtggagatcaag

SEQ ID NO: 306 - protein, 119 aa, Artificial Sequence
  source: /note="Description of Artificial Sequence: Synthetic polypeptide"
QVQLQQWGAGLLKPSETLSLTCAVYGGSFSGYYWSWIRQPPGKGLEWIGEINHRGSTNYNPSLKSRVTISVDTSKNQFSLKLSSVTAADTAVYYCTRGEEWESLFFDYWGQGTLVTVSS

SEQ ID NO: 307 - protein, 107 aa, Artificial Sequence
  source: /note="Description of Artificial Sequence: Synthetic polypeptide"
EIVLTQSPATLSLSPGERATLSCRASQSISSYLAWYQQKPGQAPRLLIYGASNRATGIPARFSGSGSGTDFTLTISSLEPEDFAVYYCQQRSNWPLTFGGGTRVEIK

SEQ ID NO: 308 - protein, 8 aa, Artificial Sequence
  source: /note="Description of Artificial Sequence: Synthetic peptide"
GGSFSGYY

SEQ ID NO: 309 - protein, 7 aa, Artificial Sequence
  source: /note="Description of Artificial Sequence: Synthetic peptide"
INHRGST

SEQ ID NO: 310 - protein, 15 aa, Artificial Sequence
  source: /note="Description of Artificial Sequence: Synthetic peptide"
CTRGEEWESLFFDYW

SEQ ID NO: 311 - protein, 6 aa, Artificial Sequence
  source: /note="Description of Artificial Sequence: Synthetic peptide"
QSISSY

SEQ ID NO: 312 - protein, 3 aa, Artificial Sequence
  source: /note="Description of Artificial Sequence: Synthetic peptide"
GAS

SEQ ID NO: 313 - protein, 11 aa, Artificial Sequence [sequence omitted]

SEQ ID NO: 314 - DNA, 366 bp, Artificial Sequence
  source: /note="Description of Artificial Sequence: Synthetic polynucleotide"
caggttcagctgcagcagtggggcgccggcctgctgagaccaagcgagaccctgtccctgacatgcgccgtgtatggcgagagcttctccggctattactggaactggatccggcagcctcccggcaagggcctggagtggatcggcgagatcaatcactccggctccaccaattacaacccatccctgaagtctcgggtgacaatcagcgtggatacaagcaagacccagttcagcctgaagctgagctccgtgacagctgccgataccgccgtgtattactgcgccagaggctgggacctgctggattggaatgactactggaatgagtactggggccaggggaccctggtgaccgtctcgagt

SEQ ID NO: 315 - DNA, 321 bp, Artificial Sequence
  source: /note="Description of Artificial Sequence: Synthetic polynucleotide"
gagatcgtgctgacccagtcccctgccaccctgtctctgtcccctggcgagcgggccaccctgtcctgtagagcttctcagtccgtgtcttcctacctggcttggtaccagcagaagccaggacaggccccaagactgctgatctatgacgcttccaatcgggctaccggcatcccagctcgctttagcggctccggctccggcaccgacttcaccctgacaatcagctccctggagccagaggattttgccgtgtattactgtcagcagaggtccaattggccactgacatttggcggcggcacaaaggttgagatcaag

SEQ ID NO: 316 - protein, 122 aa, Artificial Sequence
  source: /note="Description of Artificial Sequence: Synthetic polypeptide"
QVQLQQWGAGLLRPSETLSLTCAVYGESFSGYYWNWIRQPPGKGLEWIGEINHSGSTNYNPSLKSRVTISVDTSKTQFSLKLSSVTAADTAVYYCARGWDLLDWNDYWNEYWGQGTLVTVSS

SEQ ID NO: 317 - protein, 107 aa, Artificial Sequence; identical to SEQ ID NO: 4
  source: /note="Description of Artificial Sequence: Synthetic polypeptide"

SEQ ID NO: 318 - protein, 8 aa, Artificial Sequence
  source: /note="Description of Artificial Sequence: Synthetic peptide"
GESFSGYY

SEQ ID NO: 319 - protein, 7 aa, Artificial Sequence
  source: /note="Description of Artificial Sequence: Synthetic peptide"
INHSGST

SEQ ID NO: 320 - protein, 18 aa, Artificial Sequence
  source: /note="Description of Artificial Sequence: Synthetic peptide"
CARGWDLLDWNDYWNEYW

SEQ ID NO: 321 - protein, 6 aa, Artificial Sequence
  source: /note="Description of Artificial Sequence: Synthetic peptide"
QSVSSY

SEQ ID NO: 322 - protein, 3 aa, Artificial Sequence
  source: /note="Description of Artificial Sequence: Synthetic peptide"
DAS

SEQ ID NO: 323 - protein, 11 aa, Artificial Sequence [sequence omitted]

SEQ ID NO: 324 - DNA, 357 bp, Artificial Sequence
  source: /note="Description of Artificial Sequence: Synthetic polynucleotide"
caggttcagctgcagcagtggggcgctggcctgctgaagccctctgagaccctgtctctgacctgtgccgtgtatggcggcagcttctccggctattactggaactggatccgccagccccccggcaagggcctggagtggatcggcgagatcaaccactccggctctaccaactacaatccttctctgaagtccagggtgacaatcagcgtggacaccagcaagaaccagtttagcctgaagctgtccagcgtgacagctgccgatacagccgtgtattactgcgccagaggcgaggattggggcgagagcttctttgattactggggccaggggaccctggtgaccgtctcgagt

SEQ ID NO: 325 - DNA, 321 bp, Artificial Sequence
  source: /note="Description of Artificial Sequence: Synthetic polynucleotide"
gagatcgtgctgacccagtcccctgccaccctgtctctgtcccctggcgagcgggccaccctgagctgtcgggcctcccagtccgtgagctcctacctggcttggtatcagcagaagccaggacaggccccaagactgctgatctacgccgcttccaatcgggccaccggcatccccgccagattttccggctctggctccggcaccgatttcaccctgacaatcagctccctggagccagaggacttcgccgtgtactactgccagcagaggtctaattggccactgacatttggcggcggcaccaaggttgagatcaag

SEQ ID NO: 326 - protein, 119 aa, Artificial Sequence
  source: /note="Description of Artificial Sequence: Synthetic polypeptide"
QVQLQQWGAGLLKPSETLSLTCAVYGGSFSGYYWNWIRQPPGKGLEWIGEINHSGSTNYNPSLKSRVTISVDTSKNQFSLKLSSVTAADTAVYYCARGEDWGESFFDYWGQGTLVTVSS

SEQ ID NO: 327 - protein, 107 aa, Artificial Sequence
  source: /note="Description of Artificial Sequence: Synthetic polypeptide"
EIVLTQSPATLSLSPGERATLSCRASQSVSSYLAWYQQKPGQAPRLLIYAASNRATGIPARFSGSGSGTDFTLTISSLEPEDFAVYYCQQRSNWPLTFGGGTKVEIK

SEQ ID NO: 328 - protein, 8 aa, Artificial Sequence
  source: /note="Description of Artificial Sequence: Synthetic peptide"
GGSFSGYY

SEQ ID NO: 329 - protein, 7 aa, Artificial Sequence
  source: /note="Description of Artificial Sequence: Synthetic peptide"
INHSGST

SEQ ID NO: 330 - protein, 15 aa, Artificial Sequence
  source: /note="Description of Artificial Sequence: Synthetic peptide"
CARGEDWGESFFDYW

SEQ ID NO: 331 - protein, 6 aa, Artificial Sequence
  source: /note="Description of Artificial Sequence: Synthetic peptide"
QSVSSY

SEQ ID NO: 332 - protein, 3 aa, Artificial Sequence
  source: /note="Description of Artificial Sequence: Synthetic peptide"
AAS

SEQ ID NO: 333 - protein, 11 aa, Artificial Sequence [sequence omitted]

SEQ ID NO: 334 - DNA, 357 bp, Artificial Sequence
  source: /note="Description of Artificial Sequence: Synthetic polynucleotide"
caggttcagctggtgcagtccggcgctgaggtgaagaagcctggagcttctgtgaaggtttcctgtaaggtttccggctatagcctgaccgagatctctatgcactgggtacggcaagcccccggcaagggcctggagtggatgggcggctttgacccagaggatggcgagaccatctacgctcagaggtttcaggggcgcgtgatcatgaccgaggataccagcaccgataccgcctacatggagctgtccagcctgagatccgaggataccgccgtgtattactgcgctactggtggctggggccccaattggttcgatccttggggccaggggaccctggtgaccgtctcgagt

SEQ ID NO: 335 - DNA, 321 bp, Artificial Sequence
  source: /note="Description of Artificial Sequence: Synthetic polynucleotide"
gacatccagatgacacagtctccttcctctgtgagcgcctctgtgggcgaccgcgtgaccatcacatgccgcgcttcccaggggatctcttcctggctggcttggtaccagcagaagcccggcaaggcccccaagctgctgatctatgctgccagcagcctgcagtccggcgtgccttccaggtttagcggctccggctccggcaccgactttacactgacaatcagctccctgcagcccgaggattttgccacctattactgtcagcaggcgaattccttcccttttacattcggccctggcaccaaggttgatatcaag

SEQ ID NO: 336 - protein, 119 aa, Artificial Sequence
  source: /note="Description of Artificial Sequence: Synthetic polypeptide"
QVQLVQSGAEVKKPGASVKVSCKVSGYSLTEISMHWVRQAPGKGLEWMGGFDPEDGETIYAQRFQGRVIMTEDTSTDTAYMELSSLRSEDTAVYYCATGGWGPNWFDPWGQGTLVTVSS

SEQ ID NO: 337 - protein, 107 aa, Artificial Sequence
  source: /note="Description of Artificial Sequence: Synthetic polypeptide"
DIQMTQSPSSVSASVGDRVTITCRASQGISSWLAWYQQKPGKAPKLLIYAASSLQSGVPSRFSGSGSGTDFTLTISSLQPEDFATYYCQQANSFPFTFGPGTKVDIK

SEQ ID NO: 338 - protein, 8 aa, Artificial Sequence
  source: /note="Description of Artificial Sequence: Synthetic peptide"
GYSLTEIS

SEQ ID NO: 339 - protein, 8 aa, Artificial Sequence
  source: /note="Description of Artificial Sequence: Synthetic peptide"
FDPEDGET

SEQ ID NO: 340 - protein, 14 aa, Artificial Sequence
  source: /note="Description of Artificial Sequence: Synthetic peptide"
CATGGWGPNWFDPW

SEQ ID NO: 341 - protein, 6 aa, Artificial Sequence
  source: /note="Description of Artificial Sequence: Synthetic peptide"
QGISSW

SEQ ID NO: 342 - protein, 3 aa, Artificial Sequence
  source: /note="Description of Artificial Sequence: Synthetic peptide"
AAS

SEQ ID NO: 343 - protein, 11 aa, Artificial Sequence [sequence omitted]

SEQ ID NO: 344 - DNA, 363 bp, Artificial Sequence
  source: /note="Description of Artificial Sequence: Synthetic polynucleotide"
caggttcagctgcagcagtccggccccggcctggtgaagccaagccagaccctgtctctgacatgcgccatctccggcgacagcgtgtcctctaactccgccgcttggaattggatccggcagtctccatccagaggcctggagtggctgggcagaacctattaccggtccaagtggtacaacgattatgccgtgtccgtgaagagcagaatcaccatcaaccctgataccagcaagaaccagttcagcctgcagctgaattccgtgaccccagaggatacagccgtgtattactgtgctagggacgatgattggaatgacttcgattactggggccaggggaccctggtgacagtctcgagt

SEQ ID NO: 345 - DNA, 321 bp, Artificial Sequence
  source: /note="Description of Artificial Sequence: Synthetic polynucleotide"
gagatcgtgctgacccagtccccagctacactgtccctgtctcccggcgagcgggccaccctgagctgtagagcttcccagtccgtgtcttcctatctggcttggtatcagcagaagccaggacaggccccaaggctgctgatctacgacgcctccaatagagccaccggcatcccagctagattttctggctccggctccggcaccgatttcacactgaccatctctagcctggagccagaggattttgctgtatattactgccagcagcgcagcaactggcccctgacatttggcggcggcaccaaggttgagatcaag

SEQ ID NO: 346 - protein, 121 aa, Artificial Sequence
  source: /note="Description of Artificial Sequence: Synthetic polypeptide"
QVQLQQSGPGLVKPSQTLSLTCAISGDSVSSNSAAWNWIRQSPSRGLEWLGRTYYRSKWYNDYAVSVKSRITINPDTSKNQFSLQLNSVTPEDTAVYYCARDDDWNDFDYWGQGTLVTVSS

SEQ ID NO: 347 - protein, 107 aa, Artificial Sequence; identical to SEQ ID NO: 4
  source: /note="Description of Artificial Sequence: Synthetic polypeptide"

SEQ ID NO: 348 - protein, 9 aa, Artificial Sequence
  source: /note="Description of Artificial Sequence: Synthetic peptide"
GDSVSSNSA

SEQ ID NO: 349 - protein, 7 aa, Artificial Sequence
  source: /note="Description of Artificial Sequence: Synthetic peptide"
TYYRSKW

SEQ ID NO: 350 - protein, 13 aa, Artificial Sequence
  source: /note="Description of Artificial Sequence: Synthetic peptide"
CARDDDWNDFDYW

SEQ ID NO: 351 - protein, 6 aa, Artificial Sequence
  source: /note="Description of Artificial Sequence: Synthetic peptide"
QSVSSY

SEQ ID NO: 352 - protein, 3 aa, Artificial Sequence
  source: /note="Description of Artificial Sequence: Synthetic peptide"
DAS

SEQ ID NO: 353 - protein, 11 aa, Artificial Sequence [sequence omitted]

SEQ ID NO: 354 - DNA, 372 bp, Artificial Sequence
  source: /note="Description of Artificial Sequence: Synthetic polynucleotide"
cagctgcagctgcaggaaagcggccccggcctggtgaagccctctgagaccctgtccctgacatgcaccgtgagcggcgattccatcagctcttccagctattactggggctggatccggcagccccccggcaagggcctggagtggatcggcagcatcttctactccggcaatacatattataatccttctctgaagagcagggtgacaatcagcgtggatacctccaagaatcagtttagcctgaagctgagctccgtgacagctgccgatacagccgtgtattactgcgctagggaggacgattttctgaccgattattacggcgctttcgacatctggggccaggggacaatggtgacagtctcgagt

SEQ ID NO: 355 - DNA, 318 bp, Artificial Sequence
  source: /note="Description of Artificial Sequence: Synthetic polynucleotide"
gatatccagatgacccagtctccaagcaccctgagcgcctctgtgggcgatcgggtgaccatcacatgtcgggcttctcagtccatcagcagctggctggcttggtatcagcagaagcccggcaaggccccaaagctgctgatctacaaggcctcttccagcgagagcggcgtgccatccaggtttagcggctccggctccggcaccgagtttaccctgaccatctcttccctgcagcccgatgactttgccacctactactgtcagcagtacaattcctatctgacattcggcggcggcaccaaggttgagatcaag

SEQ ID NO: 356 - protein, 124 aa, Artificial Sequence
  source: /note="Description of Artificial Sequence: Synthetic polypeptide"
QLQLQESGPGLVKPSETLSLTCTVSGDSISSSSYYWGWIRQPPGKGLEWIGSIFYSGNTYYNPSLKSRVTISVDTSKNQFSLKLSSVTAADTAVYYCAREDDFLTDYYGAFDIWGQGTMVTVSS

SEQ ID NO: 357 - protein, 106 aa, Artificial Sequence
  source: /note="Description of Artificial Sequence: Synthetic polypeptide"
DIQMTQSPSTLSASVGDRVTITCRASQSISSWLAWYQQKPGKAPKLLIYKASSSESGVPSRFSGSGSGTEFTLTISSLQPDDFATYYCQQYNSYLTFGGGTKVEIK

SEQ ID NO: 358 - protein, 10 aa, Artificial Sequence
  source: /note="Description of Artificial Sequence: Synthetic peptide"
GDSISSSSYY

SEQ ID NO: 359 - protein, 7 aa, Artificial Sequence
  source: /note="Description of Artificial Sequence: Synthetic peptide"
IFYSGNT

SEQ ID NO: 360 - protein, 18 aa, Artificial Sequence
  source: /note="Description of Artificial Sequence: Synthetic peptide"
CAREDDFLTDYYGAFDIW

SEQ ID NO: 361 - protein, 6 aa, Artificial Sequence
  source: /note="Description of Artificial Sequence: Synthetic peptide"
QSISSW

SEQ ID NO: 362 - protein, 3 aa, Artificial Sequence
  source: /note="Description of Artificial Sequence: Synthetic peptide"
KAS

SEQ ID NO: 363 - protein, 10 aa, Artificial Sequence [sequence omitted]

SEQ ID NO: 364 - DNA, 375 bp, Artificial Sequence
  source: /note="Description of Artificial Sequence: Synthetic polynucleotide"
gaggtgcagctgctggaatccggaggaggactggtccagccaggtggatccctgcgactgagctgcgccgcttctggcttcgactttagaagctacgcaatgatgtgggtccgccaggcaccaggaaagggactggagtgggtgggagggatcaacggtgaagtcggtggctctaatacatactatgcacctgccgtcaagggaagggctactattagtcgggacaactcaaaaaataccctgtatctgcaaatgaacagtctgagggccgaggataccgccgtgtactattgcgtgaaaggtgctggcgcatgcggcatctgtaatgacgatattgatgcatggggacaggggaccctggtgacagtctcgagt

SEQ ID NO: 365 - DNA, 330 bp, Artificial Sequence
  source: /note="Description of Artificial Sequence: Synthetic polynucleotide"
agttatgagctgactcaggacccagcagtgtcagtcgccctgggccagacagtgagaatcacttgcagtggggctggttcatatgcaggctcctactattacggatggcaccagcagaagcccggacaggcacctgtgacagtcatctacgacaacgataaaaggccaagcaatattcccgaccggttctctgggtccagctctggtaacaccgcctccctgaccattactggggcccaggctgaggacgaagctgattattactgtggctctacaaacgataatgacgatggcggactgtttggctccggaactaaggtcaccgtccta

SEQ ID NO: 366 - protein, 125 aa, Artificial Sequence
  source: /note="Description of Artificial Sequence: Synthetic polypeptide"
EVQLLESGGGLVQPGGSLRLSCAASGFDFRSYAMMWVRQAPGKGLEWVGGINGEVGGSNTYYAPAVKGRATISRDNSKNTLYLQMNSLRAEDTAVYYCVKGAGACGICNDDIDAWGQGTLVTVSS

SEQ ID NO: 367 - protein, 110 aa, Artificial Sequence
  source: /note="Description of Artificial Sequence: Synthetic polypeptide"
SYELTQDPAVSVALGQTVRITCSGAGSYAGSYYYGWHQQKPGQAPVTVIYDNDKRPSNIPDRFSGSSSGNTASLTITGAQAEDEADYYCGSTNDNDDGGLFGSGTKVTVL

SEQ ID NO: 368 - protein, 8 aa, Artificial Sequence
  source: /note="Description of Artificial Sequence: Synthetic peptide"
GFDFRSYA

SEQ ID NO: 369 - protein, 10 aa, Artificial Sequence
  source: /note="Description of Artificial Sequence: Synthetic peptide"
INGEVGGSNT

SEQ ID NO: 370 - protein, 18 aa, Artificial Sequence
  source: /note="Description of Artificial Sequence: Synthetic peptide"
CVKGAGACGICNDDIDAW

SEQ ID NO: 371 - protein, 7 aa, Artificial Sequence
  source: /note="Description of Artificial Sequence: Synthetic peptide"
GSYAGSY

SEQ ID NO: 372 - protein, 3 aa, Artificial Sequence
  source: /note="Description of Artificial Sequence: Synthetic peptide"
DND

SEQ ID NO: 373 - protein, 13 aa, Artificial Sequence
  source: /note="Description of Artificial Sequence: Synthetic peptide"
CGSTNDNDDGGLF

SEQ ID NO: 374 - protein, 330 aa, Artificial Sequence
  source: /note="Description of Artificial Sequence: Synthetic polypeptide"
ASTKGPSVFPLAPSSKSTSGGTAALGCLVKDYFPEPVTVSWNSGALTSGVHTFPAVLQSSGLYSLSSVVTVPSSSLGTQTYICNVNHKPSNTKVDKRVEPKSCDKTHTCPPCPAPELLGGPSVFLFPPKPKDTLMISRTPEVTCVVVDVSHEDPEVKFNWYVDGVEVHNAKTKPREEQYNSTYRVVSVLTVLHQDWLNGKEYKCKVSNKALPAPIEKTISKAKGQPREPQVYTLPPSREEMTKNQVSLTCLVKGFYPSDIAVEWESNGQPENNYKTTPPVLDSDGSFFLYSKLTVDKSRWQQGNVFSCSVMHEALHNHYTQKSLSLSPGK

SEQ ID NO: 375 - protein, 330 aa, Artificial Sequence
  source: /note="Description of Artificial Sequence: Synthetic polypeptide"
ASTKGPSVFPLAPSSKSTSGGTAALGCLVKDYFPEPVTVSWNSGALTSGVHTFPAVLQSSGLYSLSSVVTVPSSSLGTQTYICNVNHKPSNTKVDKRVEPKSCDKTHTCPPCPAPEAAGGPSVFLFPPKPKDTLMISRTPEVTCVVVDVSHEDPEVKFNWYVDGVEVHNAKTKPREEQYNSTYRVVSVLTVLHQDWLNGKEYKCKVSNKALPAPIEKTISKAKGQPREPQVYTLPPSREEMTKNQVSLTCLVKGFYPSDIAVEWESNGQPENNYKTTPPVLDSDGSFFLYSKLTVDKSRWQQGNVFSCSVMHEALHNHYTQKSLSLSPGK

SEQ ID NO: 376 - protein, 327 aa, Artificial Sequence
  source: /note="Description of Artificial Sequence: Synthetic polypeptide"
ASTKGPSVFPLAPCSRSTSESTAALGCLVKDYFPEPVTVSWNSGALTSGVHTFPAVLQSSGLYSLSSVVTVPSSSLGTKTYTCNVDHKPSNTKVDKRVESKYGPPCPPCPAPEFLGGPSVFLFPPKPKDTLMISRTPEVTCVVVDVSQEDPEVQFNWYVDGVEVHNAKTKPREEQFNSTYRVVSVLTVLHQDWLNGKEYKCKVSNKGLPSSIEKTISKAKGQPREPQVYTLPPSQEEMTKNQVSLTCLVKGFYPSDIAVEWESNGQPENNYKTTPPVLDSDGSFFLYSRLTVDKSRWQEGNVFSCSVMHEALHNHYTQKSLSLSLGK

SEQ ID NO: 377 - protein, 326 aa, Artificial Sequence
  source: /note="Description of Artificial Sequence: Synthetic polypeptide"
ASTKGPSVFPLAPCSRSTSESTAALGCLVKDYFPEPVTVSWNSGALTSGVHTFPAVLQSSGLYSLSSVVTVPSSNFGTQTYTCNVDHKPSNTKVDKTVERKCCVECPPCPAPPVAGPSVFLFPPKPKDTLMISRTPEVTCVVVDVSHEDPEVQFNWYVDGVEVHNAKTKPREEQFNSTFRVVSVLTVVHQDWLNGKEYKCKVSNKGLPAPIEKTISKTKGQPREPQVYTLPPSREEMTKNQVSLTCLVKGFYPSDIAVEWESNGQPENNYKTTPPMLDSDGSFFLYSKLTVDKSRWQQGNVFSCSVMHEALHNHYTQKSLSLSPGK

SEQ ID NO: 378 - protein, 107 aa, Artificial Sequence [sequence omitted]

SEQ ID NO: 379 - protein, 106 aa, Artificial Sequence
  source: /note="Description of Artificial Sequence: Synthetic polypeptide"
GQPKANPTVTLFPPSSEELQANKATLVCLISDFYPGAVTVAWKADGSPVKAGVETTKPSKQSNNKYAASSYLSLTPEQWKSHRSYSCQVTHEGSTVEKTVAPTECS

SEQ ID NO: 380 - DNA, 990 bp, Artificial Sequence
  source: /note="Description of Artificial Sequence: Synthetic polynucleotide"
gcctccaccaagggcccatcggtcttccccctggcaccctcctccaagagcacctctgggggcacagcggccctgggctgcctggtcaaggactacttccccgaaccggtgacggtgtcgtggaactcaggcgccctgaccagcggcgtgcacaccttcccggctgtcctacagtcctcaggactctactccctcagcagcgtggtgaccgtgccctccagcagcttgggcacccagacctacatctgcaacgtgaatcacaagcccagcaacaccaaggtggacaagagagttgagcccaaatcttgtgacaaaactcacacatgcccaccgtgcccagcacctgaagccgccgggggaccgtcagtcttcctcttccccccaaaacccaaggacaccctcatgatctcccggacccctgaggtcacatgcgtggtggtggacgtgagccacgaagaccctgaggtcaagttcaactggtacgtggacggcgtggaggtgcataatgccaagacaaagccgcgggaggagcagtacaacagcacgtaccgtgtggtcagcgtcctcaccgtcctgcaccaggactggctgaatggcaaggagtacaagtgcaaggtctccaacaaagccctcccagcccccatcgagaaaaccatctccaaagccaaagggcagccccgagaaccacaggtgtacaccctgcccccatcccgggaggagatgaccaagaaccaggtcagcctgacctgcctggtcaaaggcttctatcccagcgacatcgccgtggagtgggagagcaatgggcagccggagaacaactacaagaccacgcctcccgtgctggactccgacggctccttcttcctctatagcaagctcaccgtggacaagagcaggtggcagcaggggaacgtcttctcatgctccgtgatgcatgaggctctgcacaaccactacacgcagaagagcctctccctgtccccgggtaaa

SEQ ID NO: 381 - DNA, 1596 bp, Artificial Sequence
  source: /note="Description of Artificial Sequence: Synthetic polynucleotide"
gcctccaccaagggcccatcggtcttccccctggcaccctcctccaagagcacctctgggggcacagcggccctgggctgcctggtcaaggactacttccccgaaccggtgacggtgtcgtggaactcaggcgccctgaccagcggcgtgcacaccttcccggctgtcctacagtcctcaggactctactccctcagcagcgtggtgaccgtgccctccagcagcttgggcacccagacctacatctgcaacgtgaatcacaagcccagcaacaccaaggtggacaagagagttggtgagaggccagcacagggagggagggtgtctgctggaagccaggctcagcgctcctgcctggacgcatcccggctatgcagtcccagtccagggcagcaaggcaggccccgtctgcctcttcacccggaggcctctgcccgccccactcatgctcagggagagggtcttctggctttttccccaggctctgggcaggcacaggctaggtgcccctaacccaggccctgcacacaaaggggcaggtgctgggctcagacctgccaagagccatatccgggaggaccctgcccctgacctaagcccaccccaaaggccaaactctccactccctcagctcggacaccttctctcctcccagattccagtaactcccaatcttctctctgcagagcccaaatcttgtgacaaaactcacacatgcccaccgtgcccaggtaagccagcccaggcctcgccctccagctcaaggcgggacaggtgccctagagtagcctgcatccagggacaggccccagccgggtgctgacacgtccacctccatctcttcctcagcacctgaagccgccgggggaccgtcagtcttcctcttccccccaaaacccaaggacaccctcatgatctcccggacccctgaggtcacatgcgtggtggtggacgtgagccacgaagaccctgaggtcaagttcaactggtacgtggacggcgtggaggtgcataatgccaagacaaagccgcgggaggagcagtacaacagcacgtaccgtgtggtcagcgtcctcaccgtcctgcaccaggactggctgaatggcaaggagtacaagtgcaaggtctccaacaaagccctcccagcccccatcgagaaaaccatctccaaagccaaaggtgggacccgtggggtgcgagggccacatggacagaggccggctcggcccaccctctgccctgagagtgaccgctgtaccaacctctgtccctacagggcagccccgagaaccacaggtgtacaccctgcccccatcccgggaggagatgaccaagaaccaggtcagcctgacctgcctggtcaaaggcttctatcccagcgacatcgccgtggagtgggagagcaatgggcagccggagaacaactacaagaccacgcctcccgtgctggactccgacggctccttcttcctctatagcaagctcaccgtggacaagagcaggtggcagcaggggaacgtcttctcatgctccgtgatgcatgaggctctgcacaaccactacacgcagaagagcctctccctgtccccgggtaaa

SEQ ID NO: 382 - DNA, 981 bp, Artificial Sequence
  source: /note="Description of Artificial Sequence: Synthetic polynucleotide"
gcttccaccaagggcccatcggtcttccccctggcgccctgctccaggagcacctccgagagcacagccgccctgggctgcctggtcaaggactacttccccgaaccggtgacggtgtcgtggaactcaggcgccctgaccagcggcgtgcacaccttcccggctgtcctacagtcctcaggactctactccctcagcagcgtggtgaccgtgccctccagcagcttgggcacgaagacctacacctgcaacgtagatcacaagcccagcaacaccaaggtggacaagagagttgagtccaaatatggtcccccatgcccaccatgcccagcacctgagttcctggggggaccatcagtcttcctgttccccccaaaacccaaggacactctcatgatctcccggacccctgaggtcacgtgcgtggtggtggacgtgagccaggaagaccccgaggtccagttcaactggtacgtggatggcgtggaggtgcataatgccaagacaaagccgcgggaggagcagttcaacagcacgtaccgtgtggtcagcgtcctcaccgtcctgcaccaggactggctgaacggcaaggagtacaagtgcaaggtctccaacaaaggcctcccgtcctccatcgagaaaaccatctccaaagccaaagggcagccccgagagccacaggtgtacaccctgcccccatcccaggaggagatgaccaagaaccaggtcagcctgacctgcctggtcaaaggcttctaccccagcgacatcgccgtggagtgggagagcaatgggcagccggagaacaactacaagaccacgcctcccgtgctggactccgacggctccttcttcctctacagcaggctcaccgtggacaagagcaggtggcaggaggggaatgtcttctcatgctccgtgatgcatgaggctctgcacaaccactacacacagaagagcctctccctgtctctgggtaaa

SEQ ID NO: 383 - DNA, 1588 bp, Artificial Sequence
  source: /note="Description of Artificial Sequence: Synthetic polynucleotide"
gcttccaccaagggcccatcggtcttccccctggcgccctgctccaggagcacctccgagagcacagccgccctgggctgcctggtcaaggactacttccccgaaccggtgacggtgtcgtggaactcaggcgccctgaccagcggcgtgcacaccttcccggctgtcctacagtcctcaggactctactccctcagcagcgtggtgaccgtgccctccagcagcttgggcacgaagacctacacctgcaacgtagatcacaagcccagcaacaccaaggtggacaagagagttggtgagaggccagcacagggagggagggtgtctgctggaagccaggctcagccctcctgcctggacgcaccccggctgtgcagccccagcccagggcagcaaggcaggccccatctgtctcctcacccggaggcctctgaccaccccactcatgctcagggagagggtcttctggatttttccaccaggctccgggcagccacaggctggatgcccctaccccaggccctgagcatacaggggcaggtgctgcgctcagacctgccaagagccatatccgggaggaccctgcccctgacctaagcccaccccaaaggccaaactctccactccctcagctcagacaccttctctcctcccagatctgagtaactcccaatcttctctctgcagagtccaaatatggtcccccatgcccaccatgcccaggtaagccaacccaggcctcgccctccagctcaaggcgggacaggtgccctagagtagcctgcatccagggacaggccccagccgggtgctgacgcatccacctccatctcttcctcagcacctgagttcctggggggaccatcagtcttcctgttccccccaaaacccaaggacactctcatgatctcccggacccctgaggtcacgtgcgtggtggtggacgtgagccaggaagaccccgaggtccagttcaactggtacgtggatggcgtggaggtgcataatgccaagacaaagccgcgggaggagcagttcaacagcacgtaccgtgtggtcagcgtcctcaccgtcctgcaccaggactggctgaacggcaaggagtacaagtgcaaggtctccaacaaaggcctcccgtcctccatcgagaaaaccatctccaaagccaaaggtgggacccacggggtgcgagggccacatggacagaggtcagctcggcccaccctctgccctgggagtgaccgctgtgccaacctctgtccctacagggcagccccgagagccacaggtgtacaccctgcccccatcccaggaggagatgaccaagaaccaggtcagcctgacctgcctggtcaaaggcttctaccccagcgacatcgccgtggagtgggagagcaatgggcagccggagaacaactacaagaccacgcctcccgtgctggactccgacggctccttcttcctctacagcaggctcaccgtggacaagagcaggtggcaggaggggaatgtcttctcatgctccgtgatgcatgaggctctgcacaaccactacacacagaagagcctctccctgtctctgggtaaa

SEQ ID NO: 384 - DNA, 978 bp, Artificial Sequence
  source: /note="Description of Artificial Sequence: Synthetic polynucleotide"
gcctccaccaagggcccatcggtcttccccctggcgccctgctccaggagcacctccgagagcacagccgccctgggctgcctggtcaaggactacttccccgaaccggtgacggtgtcgtggaactcaggcgctctgaccagcggcgtgcacaccttcccagctgtcctacagtcctcaggactctactccctcagcagcgtggtgaccgtgccctccagcaacttcggcacccagacctacacctgcaacgtagatcacaagcccagcaacaccaaggtggacaagacagttgagcgcaaatgttgtgtcgagtgcccaccgtgcccagcaccacctgtggcaggaccgtcagtcttcctcttccccccaaaacccaaggacaccctcatgatctcccggacccctgaggtcacgtgcgtggtggtggacgtgagccacgaagaccccgaggtccagttcaactggtacgtggacggcgtggaggtgcataatgccaagacaaagccacgggaggagcagttcaacagcacgttccgtgtggtcagcgtcctcaccgttgtgcaccaggactggctgaacggcaaggagtacaagtgcaaggtctccaacaaaggcctcccagcccccatcgagaaaaccatctccaaaaccaaagggcagccccgagaaccacaggtgtacaccctgcccccatcccgggaggagatgaccaagaaccaggtcagcctgacctgcctggtcaaaggcttctaccccagcgacatcgccgtggagtgggagagcaatgggcagccggagaacaactacaagaccacacctcccatgctggactccgacggctccttcttcctctacagcaagctcaccgtggacaagagcaggtggcagcaggggaacgtcttctcatgctccgtgatgcatgaggctctgcacaaccactacacgcagaagagcctctccctgtctccgggtaaa

SEQ ID NO: 385 - DNA, 1585 bp, Artificial Sequence
  source: /note="Description of Artificial Sequence: Synthetic polynucleotide"
gcctccaccaagggcccatcggtcttccccctggcgccctgctccaggagcacctccgagagcacagccgccctgggctgcctggtcaaggactacttccccgaaccggtgacggtgtcgtggaactcaggcgctctgaccagcggcgtgcacaccttcccagctgtcctacagtcctcaggactctactccctcagcagcgtggtgaccgtgccctccagcaacttcggcacccagacctacacctgcaacgtagatcacaagcccagcaacaccaaggtggacaagacagttggtgagaggccagctcagggagggagggtgtctgctggaagccaggctcagccctcctgcctggacgcaccccggctgtgcagccccagcccagggcagcaaggcaggccccatctgtctcctcacccggaggcctctgcccgccccactcatgctcagggagagggtcttctggctttttccaccaggctccaggcaggcacaggctgggtgcccctaccccaggcccttcacacacaggggcaggtgcttggctcagacctgccaaaagccatatccgggaggaccctgcccctgacctaagccgaccccaaaggccaaactgtccactccctcagctcggacaccttctctcctcccagatccgagtaactcccaatcttctctctgcagagcgcaaatgttgtgtcgagtgcccaccgtgcccaggtaagccagcccaggcctcgccctccagctcaaggcgggacaggtgccctagagtagcctgcatccagggacaggccccagctgggtgctgacacgtccacctccatctcttcctcagcaccacctgtggcaggaccgtcagtcttcctcttccccccaaaacccaaggacaccctcatgatctcccggacccctgaggtcacgtgcgtggtggtggacgtgagccacgaagaccccgaggtccagttcaactggtacgtggacggcgtggaggtgcataatgccaagacaaagccacgggaggagcagttcaacagcacgttccgtgtggtcagcgtcctcaccgttgtgcaccaggactggctgaacggcaaggagtacaagtgcaaggtctccaacaaaggcctcccagcccccatcgagaaaaccatctccaaaaccaaaggtgggacccgcggggtatgagggccacatggacagaggccggctcggcccaccctctgccctgggagtgaccgctgtgccaacctctgtccctacagggcagccccgagaaccacaggtgtacaccctgcccccatcccgggaggagatgaccaagaaccaggtcagcctgacctgcctggtcaaaggcttctaccccagcgacatcgccgtggagtgggagagcaatgggcagccggagaacaactacaagaccacacctcccatgctggactccgacggctccttcttcctctacagcaagctcaccgtggacaagagcaggtggcagcaggggaacgtcttctcatgctccgtgatgcatgaggctctgcacaaccactacacgcagaagagcctctccctgtctccgggtaaa

SEQ ID NO: 386 - DNA, 321 bp, Artificial Sequence
  source: /note="Description of Artificial Sequence: Synthetic polynucleotide"
cgtacggtggctgcaccatctgtcttcatcttcccgccatctgatgagcagttgaaatctggaactgcctctgttgtgtgcctgctgaataacttctatcccagagaggccaaagtacagtggaaggtggataacgccctccaatcgggtaactcccaggagagtgtcacagagcaggacagcaaggacagcacctacagcctcagcagcaccctgacgctgagcaaagcagactacgagaaacacaaagtctacgcctgcgaagtcacccatcagggcctgagctcgcccgtcacaaagagcttcaacaggggagagtgt

SEQ ID NO: 387 - DNA, 325 bp, Artificial Sequence
  source: /note="Description of Artificial Sequence: Synthetic polynucleotide"
cctaggtcagcccaaggccaaccccactgtcactctgttcccgccctcctctgaggagctccaagccaacaaggccacactagtgtgtctgatcagtgacttctacccgggagctgtgacagtggcctggaaggcagatggcagccccgtcaaggcgggagtggagaccaccaaaccctccaaacagagcaacaacaagtacgcggccagcagctacctgagcctgacgcccgagcagtggaagtcccacagaagctacagctgccaggtcacgcatgaagggagcaccgtggagaagacagtggcccctacagaatgttcataa

SEQ ID NO: 388 - protein, 288 aa, Homo sapiens
MQIPQAPWPVVWAVLQLGWRPGWFLDSPDRPWNPPTFSPALLVVTEGDNATFTCSFSNTSESFVLNWYRMSPSNQTDKLAAFPEDRSQPGQDCRFRVTQLPNGRDFHMSVVRARRNDSGTYLCGAISLAPKAQIKESLRAELRVTERRAEVPTAHPSPSPRPAGQFQTLVVGVVGGLLGSLVLLVWVLAVICSRAARGTIGARRTGQPLKEDPSAVPVFSVDYGELDFQWREKTPEPPVPCVPEQTEYATIVFPSGMGTSSPARRGSADGPRSAQPLRPEDGHCSWPL

SEQ ID NO: 389 - protein, 301 aa, Homo sapiens
MFSHLPFDCVLLLLLLLLTRSSEVEYRAEVGQNAYLPCFYTPAAPGNLVPVCWGKGACPVFECGNVVLRTDERDVNYWTSRYWLNGDFRKGDVSLTIENVTLADSGIYCCRIQIPGIMNDEKFNLKLVIKPAKVTPAPTRQRDFTAAFPRMLTTRGHGPAETQTLGSLPDINLTQISTLANELRDSRLANDLRDSGATIRIGIYIGAGICAGLALALIFGALIFKWYSHSKEKIQNLSLISLANLPPSGLANAVAEGIRSEENIYTIEENVYEVEEPNEYYCYVSSRQQPSQPLGCRFAMP

SEQ ID NO: 390 - protein, 525 aa, Homo sapiens
MWEAQFLGLLFLQPLWVAPVKPLQPGAEVPVVWAQEGAPAQLPCSPTIPLQDLSLLRRAGVTWQHQPDSGPPAAAPGHPLAPGPHPAAPSSWGPRPRRYTVLSVGPGGLRSGRLPLQPRVQLDERGRQRGDFSLWLRPARRADAGEYRAAVHLRDRALSCRLRLRLGQASMTASPPGSLRASDWVILNCSFSRPDRPASVHWFRNRGQGRVPVRESPHHHLAESFLFLPQVSPMDSGPWGCILTYRDGFNVSIMYNLTVLGLEPPTPLTVYAGAGSRVGLPCRLPAGVGTRSFLTAKWTPPGGGPDLLVTGDNGDFTLRLEDVSQAQAGTYTCHIHLQEQQLNATVTLAIITVTPKSFGSPGSLGKLLCEVTPVSGQERFVWSSLDTPSQRSFSGPWLEAQEAQLLSQPWQCQLYQGERLLGAAVYFTELSSPGAQRSGRAPGALPAGHLLLFLILGVLSLLLLVTGAFGFHLWRRQWRPRRFSALEQGIHPPQAQSKIEELEQEPEPEPEPEPEPEPEPEPEQL

SEQ ID NO: 391 - DNA, 321 bp, Artificial Sequence
  source: /note="Description of Artificial Sequence: Synthetic polynucleotide"
gctagcctcttacgagctgactcagccaccttccgtgtccgtgtccccaggacagaccgcaagaatcacatgcagtggcggatccagctactcatatgggtggttccagcagaagcctggtcaggcccccgtgacagtcatctatgagagcaacaataggccttctgacattccagaacggtttagtggctctagttcaggaaccacagtgactctgaccatcagcggggtccaggccgaggacgaagctgattactattgtggcaacgctgattccagctctggaattttcgggtccggtacaaaagtgactgtcctagg

SEQ ID NO: 392 - protein, 104 aa, Artificial Sequence
  source: /note="Description of Artificial Sequence: Synthetic polypeptide"
SYELTQPPSVSVSPGQTARITCSGGSSYSYGWFQQKPGQAPVTVIYESNNRPSDIPERFSGSSSGTTVTLTISGVQAEDEADYYCGNADSSSGIFGSGTKVTVL

SEQ ID NO: 393 - protein, 4 aa, Artificial Sequence
  source: /note="Description of Artificial Sequence: Synthetic peptide"
SSYS

SEQ ID NO: 394 - protein, 3 aa, Artificial Sequence
  source: /note="Description of Artificial Sequence: Synthetic peptide"
ESN

SEQ ID NO: 395 - protein, 11 aa, Artificial Sequence
  source: /note="Description of Artificial Sequence: Synthetic peptide"
CGNADSSSGIF

SEQ ID NO: 396 - protein, 15 aa, Artificial Sequence
  source: /note="Description of Artificial Sequence: Synthetic peptide"
GGGGSGGGGSGGGGS

SEQ ID NO: 397 - protein, 6 aa, Homo sapiens
KIEELE